European Patent Application EP 4 567 114 A1, published June 11, 2025. Title: Shortened polycystin-1 polypeptide and use thereof. Applicant: 大塚製薬株式会社. The sequence listing filed with the application follows.

SEQUENCE LISTING (60 sequences)

SEQ ID NO: 1 - protein, 4303 aa, Homo sapiens
MPPAAPARLALALGLGLWLGALAGGPGRGCGPCEPPCLCGPAPGAACRVNCSGRGLRTLGPALRIPADATALDVSHNLLRALDVGLLANLSALAELDISNNKISTLEEGIFANLFNLSEINLSGNPFECDCGLAWLPRWAEEQQVRVVQPEAATCAGPGSLAGQPLLGIPLLDSGCGEEYVACLPDNSSGTVAAVSFSAAHEGLLQPEACSAFCFSTGQGLAALSEQGWCLCGAAQPSSASFACLSLCSGPPPPPAPTCRGPTLLQHVFPASPGATLVGPHGPLASGQLAAFHIAAPLPVTATRWDFGDGSAEVDAAGPAASHRYVLPGRYHVTAVLALGAGSALLGTDVQVEAAPAALELVCPSSVQSDESLDLSIQNRGGSGLEAAYSIVALGEEPARAVHPLCPSDTEIFPGNGHCYRLVVEKAAWLQAQEQCQAWAGAALAMVDSPAVQRFLVSRVTRSLDVWIGFSTVQGVEVGPAPQGEAFSLESCQNWLPGEPHPATAEHCVRLGPTGWCNTDLCSAPHSYVCELQPGGPVQDAENLLVGAPSGDLQGPLTPLAQQDGLSAPHEPVEVMVFPGLRLSREAFLTTAEFGTQELRRPAQLRLQVYRLLSTAGTPENGSEPESRSPDNRTQLAPACMPGGRWCPGANICLPLDASCHPQACANGCTSGPGLPGAPYALWREFLFSVPAGPPAQYSVTLHGQDVLMLPGDLVGLQHDAGPGALLHCSPAPGHPGPQAPYLSANASSWLPHLPAQLEGTWACPACALRLLAATEQLTVLLGLRPNPGLRLPGRYEVRAEVGNGVSRHNLSCSFDVVSPVAGLRVIYPAPRDGRLYVPTNGSALVLQVDSGANATATARWPGGSVSARFENVCPALVATFVPGCPWETNDTLFSVVALPWLSEGEHVVDVVVENSASRANLSLRVTAEEPICGLRATPSPEARVLQGVLVRYSPVVEAGSDMVFRWTINDKQSLTFQNVVFNVIYQSAAVFKLSLTASNHVSNVTVNYNVTVERMNRMQGLQVSTVPAVLSPNATLALTAGVLVDSAVEVAFLWTFGDGEQALHQFQPPYNESFPVPDPSVAQVLVEHNVMHTYAAPGEYLLTVLASNAFENLTQQVPVSVRASLPSVAVGVSDGVLVAGRPVTFYPHPLPSPGGVLYTWDFGDGSPVLTQSQPAANHTYASRGTYHVRLEVNNTVSGAAAQADVRVFEELRGLSVDMSLAVEQGAPVVVSAAVQTGDNITWTFDMGDGTVLSGPEATVEHVYLRAQNCTVTVGAASPAGHLARSLHVLVFVLEVLRVEPAACIPTQPDARLTAYVTGNPAHYLFDWTFGDGSSNTTVRGCPTVTHNFTRSGTFPLALVLSSRVNRAHYFTSICVEPEVGNVTLQPERQFVQLGDEAWLVACAWPPFPYRYTWDFGTEEAAPTRARGPEVTFIYRDPGSYLVTVTASNNISAANDSALVEVQEPVLVTSIKVNGSLGLELQQPYLFSAVGRGRPASYLWDLGDGGWLEGPEVTHAYNSTGDFTVRVAGWNEVSRSEAWLNVTVKRRVRGLVVNASRTVVPLNGSVSFSTSLEAGSDVRYSWVLCDRCTPIPGGPTISYTFRSVGTFNIIVTAENEVGSAQDSIFVYVLQLIEGLQVVGGGRYFPTNHTVQLQAVVRDGTNVSYSWTAWRDRGPALAGSGKGFSLTVLEAGTYHVQLRATNMLGSAWADCTMDFVEPVGWLMVAASPNPAAVNTSVTLSAELAGGSGVVYTWSLEEGLSWETSEPFTTHSFPTPGLHLVTMTAGNPLGSANATVEVDVQVPVSGLSIRASEPGGSFVAAGSSVPFWGQLATGTNVSWCWAVPGGSSKRGPHVTMVFPDAGTFSIRLNASNAVSWVSATYNLTAEEPIVGLVLWASSKVVAPGQLVHFQILLAAGSAVTFRLQVGGANPEVLPGPRFSHSFPRVGDHVVSVRGKNHVSWAQAQVRIVVLEAVSGLQVPNCCEPGIATGTERNFTARVQRGSRVAYAWYFSLQKVQGDSLVILSGRDVTYTPVAAGLLEIQVRAFNALGSENRTLVLEVQDAVQYVALQSGPCFTNRSAQFEAATSPSPRRVAYHWDFGDGSPGQDTDEPRAEHSYLRPGDYRVQVNASNLVSFFVAQATVTVQVLACREPEVDVVLPLQVLMRRSQRNYLEAHVDLRDCVTYQTEYRWEVYRTASCQRPGRPARVALPGVDVSRPRLVLPRLALPVGHYCFVFVVSFGDTPLTQSIQANVTVAPERLVPIIEGGSYRVWSDTRDLVLDGSESYDPNLEDGDQTPLSFHWACVASTQREAGGCALNFGPRGSSTVTIPRERLAAGVEYTFSLTVWKAGRKEEATNQTVLIRSGRVPIVSLECVSCKAQAVYEVSRSSYVYLEGRCLNCSSGSKRGRWAARTFSNKTLVLDETTTSTGSAGMRLVLRRGVLRDGEGYTFTLTVLGRSGEEEGCASIRLSPNRPPLGGSCRLFPLGAVHALTTKVHFECTGWHDAEDAGAPLVYALLLRRCRQGHCEEFCVYKGSLSSYGAVLPPGFRPHFEVGLAVVVQDQLGAAVVALNRSLAITLPEPNGSATGLTVWLHGLTASVLPGLLRQADPQHVIEYSLALVTVLNEYERALDVAAEPKHERQHRAQIRKNITETLVSLRVHTVDDIQQIAAALAQCMGPSRELVCRSCLKQTLHKLEAMMLILQAETTAGTVTPTAIGDSILNITGDLIHLASSDVRAPQPSELGAESPSRMVASQAYNLTSALMRILMRSRVLNEEPLTLAGEEIVAQGKRSDPRSLLCYGGAPGPGCHFSIPEAFSGALANLSDVVQLIFLVDSNPFPFGYISNYTVSTKVASMAFQTQAGAQIPIERLASERAITVKVPNNSDWAARGHRSSANSANSVVVQPQASVGAVVTLDSSNPAAGLHLQLNYTLLDGHYLSEEPEPYLAVYLHSEPRPNEHNCSASRRIRPESLQGADHRPYTFFISPGSRDPAGSYHLNLSSHFRWSALQVSVGLYTSLCQYFSEEDMVWRTEGLLPLEETSPRQAVCLTRHLTAFGASLFVPPSHVRFVFPEPTADVNYIVMLTCAVCLVTYMVMAAILHKLDQLDASRGRAIPFCGQRGRFKYEILVKTGWGRGSGTTAHVGIMLYGVDSRSGHRHLDGDRAFHRNSLDIFRIATPHSLGSVWKIRVWHDNKGLSPAWFLQHVIVRDLQTARSAFFLVNDWLSVETEANGGLVEKEVLAASDAALLRFRRLLVAELQRGFFDKHIWLSIWDRPPRSRFTRIQRATCCVLLICLFLGANAVWYGAVGDSAYSTGHVSRLSPLSVDTVAVGLVSSVVVYPVYLAILFLFRMSRSKVAGSPSPTPAGQQVLDIDSCLDSSVLDSSFLTFSGLHAEQAFVGQMKSDLFLDDSKSLVCWPSGEGTLSWPDLLSDPSIVGSNLRQLARGQAGHGLGPEEDGFSLASPYSPAKSFSASDEDLIQQVLAEGVSSPAPTQDTHMETDLLSSLSSTPGEKTETLALQRLGELGPPSPGLNWEQPQAARLSRTGLVEGLRKRLLPAWCASLAHGLSLLLVAVAVAVSGWVGASFPPGVSVAWLLSSSASFLASFLGWEPLKVLLEALYFSLVAKRLHPDEDDTLVESPAVTPVSARVPRVRPPHGFALFLAKEEARKVKRLHGMLRSLLVYMLFLLVTLLASYGDASCHGHAYRLQSAIKQELHSRAFLAITRSEELWPWMAHVLLPYVHGNQSSPELGPPRLRQVRLQEALYPDPPGPRVHTCSAAGGFSTSDYDVGWESPHNGSGTWAYSAPDLLGAWSWGSCAVYDSGGYVQELGLSLEESRDRLRFLQLHNWLDNRSRAVFLELTRYSPAVGLHAAVTLRLEFPAAGRALAALSVRPFALRRLSAGLSLPLLTSVCLLLFAVHFAVAEARTWHREGRWRVLRLGAWARWLLVALTAATALVRLAQLGAADRQWTRFVRGRPRRFTSFDQVAQLSSAARGLAASLLFLLLVKAAQQLRFVRQWSVFGKTLCRALPELLGVTLGLVVLGVAYAQLAILLVSSCVDSLWSVAQALLVLCPGTGLSTLCPAESWHLSPLLCVGLWALRLWGALRLGAVILRWRYHALRGELYRPAWEPQDYEMVELFLRRLRLWMGLSKVKEFRHKVRFEGMEPLPSRSSRGSKVSPDVPPPSAGSDASHPSTSSSQLDGLSVSLGRLGTRCEPEPSRLQAVFEALLTQFDRLNQATEDVYQLEQQLHSLQGRRSSRAPAGSSRGPSPGLRPALPSRLARASRGVDLATGPSRTPLRAKNKVHPSST

SEQ ID NO: 2 - DNA, 12912 bp, Homo sapiens
  source 1..12912: mol_type = other DNA
atgccgcccgccgcgcccgcccgcctggcgctggccctgggcctgggcctgtggctcggggcgctggcggggggccccgggcgcggctgcgggccctgcgagcccccctgcctctgcggcccagcgcccggcgccgcctgccgcgtcaactgctcgggccgcgggctgcggacgctcggtcccgcgctgcgcatccccgcggacgccacagcgctagacgtctcccacaacctgctccgggcgctggacgttgggctcctggcgaacctctcggcgctggcagagctggatataagcaacaacaagatttctacgttagaagaaggaatatttgctaatttatttaatttaagtgaaataaacctgagtgggaacccgtttgagtgtgactgtggcctggcgtggctgccgcgatgggcggaggagcagcaggtgcgggtggtgcagcccgaggcagccacgtgtgctgggcctggctccctggctggccagcctctgcttggcatccccttgctggacagtggctgtggtgaggagtatgtcgcctgcctccctgacaacagctcaggcaccgtggcagcagtgtccttttcagctgcccacgaaggcctgcttcagccagaggcctgcagcgccttctgcttctccaccggccagggcctcgcagccctctcggagcagggctggtgcctgtgtggggcggcccagccctccagtgcctcctttgcctgcctgtccctctgctccggccccccgccacctcctgcccccacctgtaggggccccaccctcctccagcacgtcttccctgcctccccaggggccaccctggtggggccccacggacctctggcctctggccagctagcagccttccacatcgctgccccgctccctgtcactgccacacgctgggacttcggagacggctccgccgaggtggatgccgctgggccggctgcctcgcatcgctatgtgctgcctgggcgctatcacgtgacggccgtgctggccctgggggccggctcagccctgctggggacagacgtgcaggtggaagcggcacctgccgccctggagctcgtgtgcccgtcctcggtgcagagtgacgagagccttgacctcagcatccagaaccgcggtggttcaggcctggaggccgcctacagcatcgtggccctgggcgaggagccggcccgagcggtgcacccgctctgcccctcggacacggagatcttccctggcaacgggcactgctaccgcctggtggtggagaaggcggcctggctgcaggcgcaggagcagtgtcaggcctgggccggggccgccctggcaatggtggacagtcccgccgtgcagcgcttcctggtctcccgggtcaccaggagcctagacgtgtggatcggcttctcgactgtgcagggggtggaggtgggcccagcgccgcagggcgaggccttcagcctggagagctgccagaactggctgcccggggagccacacccagccacagccgagcactgcgtccggctcgggcccaccgggtggtgtaacaccgacctgtgctcagcgccgcacagctacgtctgcgagctgcagcccggaggcccagtgcaggatgccgagaacctcctcgtgggagcgcccagtggggacctgcagggacccctgacgcctctggcacagcaggacggcctctcagccccgcacgagcccgtggaggtcatggtattcccgggcctgcgtctgagccgtgaagccttcctcaccacggccgaatttgggacccaggagctccggcggcccgcccagctgcggctgcaggtgtaccggctcctcagcacagcagggaccccggagaacggcagcgagcctgagagcaggtccccggacaacaggacccagctggcccccgcgtgcatgccagggggacgctggtgccctggagccaacatctgcttgccgctggacgcctcctgccacccccaggcctgcgccaatggctgcacgtcagggccagggctacccggggccccctatgcgctatggagagagttcctcttctccgttcccgcggggccccccgcgcagtactcggtcaccctccacggccaggatgtcctcatgctccctggtgacctcgttggcttgcagcacgacgctggccctggcgccctcctgcactgctcgccggctcccggccaccctggtccccaggccccgtacctctccgccaacgcctcgtcatggctgccccacttgccagcccagctggagggcacttgggcctgccctgcctgtgccctgcggctgcttgcagccacggaacagctcaccgtgctgctgggcttgaggcccaaccctggactgcggctgcctgggcgctatgaggtccgggcagaggtgggcaatggcgtgtccaggcacaacctctcctgcagctttgacgtggtctccccagtggctgggctgcgggtcatctaccctgccccccgcgacggccgcctctacgtgcccaccaacggctcagccttggtgctccaggtggactctggtgccaacgccacggccacggctcgctggcctgggggcagtgtcagcgcccgctttgagaatgtctgccctgccctggtggccaccttcgtgcccggctgcccctgggagaccaacgataccctgttctcagtggtagcactgccgtggctcagtgagggggagcacgtggtggacgtggtggtggaaaacagcgccagccgggccaacctcagcctgcgggtgacggcggaggagcccatctgtggcctccgcgccacgcccagccccgaggcccgtgtactgcagggagtcctagtgaggtacagccccgtggtggaggccggctcggacatggtcttccggtggaccatcaacgacaagcagtccctgaccttccagaacgtggtcttcaatgtcatttatcagagcgcggcggtcttcaagctctcactgacggcctccaaccacgtgagcaacgtcaccgtgaactacaacgtaaccgtggagcggatgaacaggatgcagggtctgcaggtctccacagtgccggccgtgctgtcccccaatgccacgctagcactgacggcgggcgtgctggtggactcggccgtggaggtggccttcctgtggacctttggggatggggagcaggccctccaccagttccagcctccgtacaacgagtccttcccggttccagacccctcggtggcccaggtgctggtggagcacaatgtcatgcacacctacgctgccccaggtgagtacctcctgaccgtgctggcatctaatgccttcgagaacctgacgcagcaggtgcctgtgagcgtgcgcgcctccctgccctccgtggctgtgggtgtgagtgacggcgtcctggtggccggccggcccgtcaccttctacccgcacccgctgccctcgcctgggggtgttctttacacgtgggacttcggggacggctcccctgtcctgacccagagccagccggctgccaaccacacctatgcctcgaggggcacctaccacgtgcgcctggaggtcaacaacacggtgagcggtgcggcggcccaggcggatgtgcgcgtctttgaggagctccgcggactcagcgtggacatgagcctggccgtggagcagggcgcccccgtggtggtcagcgccgcggtgcagacgggcgacaacatcacgtggaccttcgacatgggggacggcaccgtgctgtcgggcccggaggcaacagtggagcatgtgtacctgcgggcacagaactgcacagtgaccgtgggtgcggccagccccgccggccacctggcccggagcctgcacgtgctggtcttcgtcctggaggtgctgcgcgttgaacccgccgcctgcatccccacgcagcctgacgcgcggctcacggcctacgtcaccgggaacccggcccactacctcttcgactggaccttcggggatggctcctccaacacgaccgtgcgggggtgcccgacggtgacacacaacttcacgcggagcggcacgttccccctggcgctggtgctgtccagccgcgtgaacagggcgcattacttcaccagcatctgcgtggagccagaggtgggcaacgtcaccctgcagccagagaggcagtttgtgcagctcggggacgaggcctggctggtggcatgtgcctggcccccgttcccctaccgctacacctgggactttggcaccgaggaagccgcccccacccgtgccaggggccctgaggtgacgttcatctaccgagacccaggctcctatcttgtgacagtcaccgcgtccaacaacatctctgctgccaatgactcagccctggtggaggtgcaggagcccgtgctggtcaccagcatcaaggtcaatggctcccttgggctggagctgcagcagccgtacctgttctctgctgtgggccgtgggcgccccgccagctacctgtgggatctgggggacggtgggtggctcgagggtccggaggtcacccacgcttacaacagcacaggtgacttcaccgttagggtggccggctggaatgaggtgagccgcagcgaggcctggctcaatgtgacggtgaagcggcgcgtgcgggggctcgtcgtcaatgcaagccgcacggtggtgcccctgaatgggagcgtgagcttcagcacgtcgctggaggccggcagtgatgtgcgctattcctgggtgctctgtgaccgctgcacgcccatccctgggggtcctaccatctcttacaccttccgctccgtgggcaccttcaatatcatcgtcacggctgagaacgaggtgggctccgcccaggacagcatcttcgtctatgtcctgcagctcatagaggggctgcaggtggtgggcggtggccgctacttccccaccaaccacacggtacagctgcaggccgtggttagggatggcaccaacgtctcctacagctggactgcctggagggacaggggcccggccctggccggcagcggcaaaggcttctcgctcaccgtgctcgaggccggcacctaccatgtgcagctgcgggccaccaacatgctgggcagcgcctgggccgactgcaccatggacttcgtggagcctgtggggtggctgatggtggccgcctccccgaacccagctgccgtcaacacaagcgtcaccctcagtgccgagctggctggtggcagtggtgtcgtatacacttggtccttggaggaggggctgagctgggagacctccgagccatttaccacccatagcttccccacacccggcctgcacttggtcaccatgacggcagggaacccgctgggctcagccaacgccaccgtggaagtggatgtgcaggtgcctgtgagtggcctcagcatcagggccagcgagcccggaggcagcttcgtggcggccgggtcctctgtgcccttttgggggcagctggccacgggcaccaatgtgagctggtgctgggctgtgcccggcggcagcagcaagcgtggccctcatgtcaccatggtcttcccggatgctggcaccttctccatccggctcaatgcctccaacgcagtcagctgggtctcagccacgtacaacctcacggcggaggagcccatcgtgggcctggtgctgtgggccagcagcaaggtggtggcgcccgggcagctggtccattttcagatcctgctggctgccggctcagctgtcaccttccgcctgcaggtcggcggggccaaccccgaggtgctccccgggccccgtttctcccacagcttcccccgcgtcggagaccacgtggtgagcgtgcggggcaaaaaccacgtgagctgggcccaggcgcaggtgcgcatcgtggtgctggaggccgtgagtgggctgcaggtgcccaactgctgcgagcctggcatcgccacgggcactgagaggaacttcacagcccgcgtgcagcgcggctctcgggtcgcctacgcctggtacttctcgctgcagaaggtccagggcgactcgctggtcatcctgtcgggccgcgacgtcacctacacgcccgtggccgcggggctgttggagatccaggtgcgcgccttcaacgccctgggcagtgagaaccgcacgctggtgctggaggttcaggacgccgtccagtatgtggccctgcagagcggcccctgcttcaccaaccgctcggcgcagtttgaggccgccaccagccccagcccccggcgtgtggcctaccactgggactttggggatgggtcgccagggcaggacacagatgagcccagggccgagcactcctacctgaggcctggggactaccgcgtgcaggtgaacgcctccaacctggtgagcttcttcgtggcgcaggccacggtgaccgtccaggtgctggcctgccgggagccggaggtggacgtggtcctgcccctgcaggtgctgatgcggcgatcacagcgcaactacttggaggcccacgttgacctgcgcgactgcgtcacctaccagactgagtaccgctgggaggtgtatcgcaccgccagctgccagcggccggggcgcccagcgcgtgtggccctgcccggcgtggacgtgagccggcctcggctggtgctgccgcggctggcgctgcctgtggggcactactgctttgtgtttgtcgtgtcatttggggacacgccactgacacagagcatccaggccaatgtgacggtggcccccgagcgcctggtgcccatcattgagggtggctcataccgcgtgtggtcagacacacgggacctggtgctggatgggagcgagtcctacgaccccaacctggaggacggcgaccagacgccgctcagtttccactgggcctgtgtggcttcgacacagagggaggctggcgggtgtgcgctgaactttgggccccgcgggagcagcacggtcaccattccacgggagcggctggcggctggcgtggagtacaccttcagcctgaccgtgtggaaggccggccgcaaggaggaggccaccaaccagacggtgctgatccggagtggccgggtgcccattgtgtccttggagtgtgtgtcctgcaaggcacaggccgtgtacgaagtgagccgcagctcctacgtgtacttggagggccgctgcctcaattgcagcagcggctccaagcgagggcggtgggctgcacgtacgttcagcaacaagacgctggtgctggatgagaccaccacatccacgggcagtgcaggcatgcgactggtgctgcggcggggcgtgctgcgggacggcgagggatacaccttcacgctcacggtgctgggccgctctggcgaggaggagggctgcgcctccatccgcctgtcccccaaccgcccgccgctggggggctcttgccgcctcttcccactgggcgctgtgcacgccctcaccaccaaggtgcacttcgaatgcacgggctggcatgacgcggaggatgctggcgccccgctggtgtacgccctgctgctgcggcgctgtcgccagggccactgcgaggagttctgtgtctacaagggcagcctctccagctacggagccgtgctgcccccgggtttcaggccacacttcgaggtgggcctggccgtggtggtgcaggaccagctgggagccgctgtggtcgccctcaacaggtctttggccatcaccctcccagagcccaacggcagcgcaacggggctcacagtctggctgcacgggctcaccgctagtgtgctcccagggctgctgcggcaggccgatccccagcacgtcatcgagtactcgttggccctggtcaccgtgctgaacgagtacgagcgggccctggacgtggcggcagagcccaagcacgagcggcagcaccgagcccagatacgcaagaacatcacggagactctggtgtccctgagggtccacactgtggatgacatccagcagatcgctgctgcgctggcccagtgcatggggcccagcagggagctcgtatgccgctcgtgcctgaagcagacgctgcacaagctggaggccatgatgctcatcctgcaggcagagaccaccgcgggcaccgtgacgcccaccgccatcggagacagcatcctcaacatcacaggagacctcatccacctggccagctcggacgtgcgggcaccacagccctcagagctgggagccgagtcaccatctcggatggtggcgtcccaggcctacaacctgacctctgccctcatgcgcatcctcatgcgctcccgcgtgctcaacgaggagcccctgacgctggcgggcgaggagatcgtggcccagggcaagcgctcggacccgcggagcctgctgtgctatggcggcgccccagggcctggctgccacttctccatccccgaggctttcagcggggccctggccaacctcagtgacgtggtgcagctcatctttctggtggactccaatccctttccctttggctatatcagcaactacaccgtctccaccaaggtggcctcgatggcattccagacacaggccggcgcccagatccccatcgagcggctggcctcagagcgcgccatcaccgtgaaggtgcccaacaactcggactgggctgcccggggccaccgcagctccgccaactccgccaactccgttgtggtccagccccaggcctccgtcggtgctgtggtcaccctggacagcagcaaccctgcggccgggctgcatctgcagctcaactatacgctgctggacggccactacctgtctgaggaacctgagccctacctggcagtctacctacactcggagccccggcccaatgagcacaactgctcggctagcaggaggatccgcccagagtcactccagggtgctgaccaccggccctacaccttcttcatttccccggggagcagagacccagcggggagttaccatctgaacctctccagccacttccgctggtcggcgctgcaggtgtccgtgggcctgtacacgtccctgtgccagtacttcagcgaggaggacatggtgtggcggacagaggggctgctgcccctggaggagacctcgccccgccaggccgtctgcctcacccgccacctcaccgccttcggcgccagcctcttcgtgcccccaagccatgtccgctttgtgtttcctgagccgacagcggatgtaaactacatcgtcatgctgacatgtgctgtgtgcctggtgacctacatggtcatggccgccatcctgcacaagctggaccagttggatgccagccggggccgcgccatccctttctgtgggcagcggggccgcttcaagtacgagatcctcgtcaagacaggctggggccggggctcaggtaccacggcccacgtgggcatcatgctgtatggggtggacagccggagcggccaccggcacctggacggcgacagagccttccaccgcaacagcctggacatcttccggatcgccaccccgcacagcctgggtagcgtgtggaagatccgagtgtggcacgacaacaaagggctcagccctgcctggttcctgcagcacgtcatcgtcagggacctgcagacggcacgcagcgccttcttcctggtcaatgactggctttcggtggagacggaggccaacgggggcctggtggagaaggaggtgctggccgcgagcgacgcagcccttttgcgcttccggcgcctgctggtggctgagctgcagcgtggcttctttgacaagcacatctggctctccatatgggaccggccgcctcgtagccgtttcactcgcatccagagggccacctgctgcgttctcctcatctgcctcttcctgggcgccaacgccgtgtggtacggggctgttggcgactctgcctacagcacggggcatgtgtccaggctgagcccgctgagcgtcgacacagtcgctgttggcctggtgtccagcgtggttgtctatcccgtctacctggccatcctttttctcttccggatgtcccggagcaaggtggctgggagcccgagccccacacctgccgggcagcaggtgctggacatcgacagctgcctggactcgtccgtgctggacagctccttcctcacgttctcaggcctccacgctgagcaggcctttgttggacagatgaagagtgacttgtttctggatgattctaagagtctggtgtgctggccctccggcgagggaacgctcagttggccggacctgctcagtgacccgtccattgtgggtagcaatctgcggcagctggcacggggccaggcgggccatgggctgggcccagaggaggacggcttctccctggccagcccctactcgcctgccaaatccttctcagcatcagatgaagacctgatccagcaggtccttgccgagggggtcagcagcccagcccctacccaagacacccacatggaaacggacctgctcagcagcctgtccagcactcctggggagaagacagagacgctggcgctgcagaggctgggggagctggggccacccagcccaggcctgaactgggaacagccccaggcagcgaggctgtccaggacaggactggtggagggtctgcggaagcgcctgctgccggcctggtgtgcctccctggcccacgggctcagcctgctcctggtggctgtggctgtggctgtctcagggtgggtgggtgcgagcttccccccgggcgtgagtgttgcgtggctcctgtccagcagcgccagcttcctggcctcattcctcggctgggagccactgaaggtcttgctggaagccctgtacttctcactggtggccaagcggctgcacccggatgaagatgacaccctggtagagagcccggctgtgacgcctgtgagcgcacgtgtgccccgcgtacggccaccccacggctttgcactcttcctggccaaggaagaagcccgcaaggtcaagaggctacatggcatgctgcggagcctcctggtgtacatgctttttctgctggtgaccctgctggccagctatggggatgcctcatgccatgggcacgcctaccgtctgcaaagcgccatcaagcaggagctgcacagccgggccttcctggccatcacgcggtctgaggagctctggccatggatggcccacgtgctgctgccctacgtccacgggaaccagtccagcccagagctggggcccccacggctgcggcaggtgcggctgcaggaagcactctacccagaccctcccggccccagggtccacacgtgctcggccgcaggaggcttcagcaccagcgattacgacgttggctgggagagtcctcacaatggctcggggacgtgggcctattcagcgccggatctgctgggggcatggtcctggggctcctgtgccgtgtatgacagcgggggctacgtgcaggagctgggcctgagcctggaggagagccgcgaccggctgcgcttcctgcagctgcacaactggctggacaacaggagccgcgctgtgttcctggagctcacgcgctacagcccggccgtggggctgcacgccgccgtcacgctgcgcctcgagttcccggcggccggccgcgccctggccgccctcagcgtccgcccctttgcgctgcgccgcctcagcgcgggcctctcgctgcctctgctcacctcggtgtgcctgctgctgttcgccgtgcacttcgccgtggccgaggcccgtacttggcacagggaagggcgctggcgcgtgctgcggctcggagcctgggcgcggtggctgctggtggcgctgacggcggccacggcactggtacgcctcgcccagctgggtgccgctgaccgccagtggacccgtttcgtgcgcggccgcccgcgccgcttcactagcttcgaccaggtggcgcagctgagctccgcagcccgtggcctggcggcctcgctgctcttcctgcttttggtcaaggctgcccagcagctacgcttcgtgcgccagtggtccgtctttggcaagacattatgccgagctctgccagagctcctgggggtcaccttgggcctggtggtgctcggggtagcctacgcccagctggccatcctgctcgtgtcttcctgtgtggactccctctggagcgtggcccaggccctgttggtgctgtgccctgggactgggctctctaccctgtgtcctgccgagtcctggcacctgtcacccctgctgtgtgtggggctctgggcactgcggctgtggggcgccctacggctgggggctgttattctccgctggcgctaccacgccttgcgtggagagctgtaccggccggcctgggagccccaggactacgagatggtggagttgttcctgcgcaggctgcgcctctggatgggcctcagcaaggtcaaggagttccgccacaaagtccgctttgaagggatggagccgctgccctctcgctcctccaggggctccaaggtatccccggatgtgcccccacccagcgctggctccgatgcctcgcacccctccacctcctccagccagctggatgggctgagcgtgagcctgggccggctggggacaaggtgtgagcctgagccctcccgcctccaagccgtgttcgaggccctgctcacccagtttgaccgactcaaccaggccacagaggacgtctaccagctggagcagcagctgcacagcctgcaaggccgcaggagcagccgggcgcccgccggatcttcccgtggcccatccccgggcctgcggccagcactgcccagccgccttgcccgggccagtcggggtgtggacctggccactggccccagcaggacaccccttcgggccaagaacaaggtccaccccagcagcacttaa

SEQ ID NO: 3 - protein, 202 aa, synthetic construct
GAVILRWRYHALRGELYRPAWEPQDYEMVELFLRRLRLWMGLSKVKEFRHKVRFEGMEPLPSRSSRGSKVSPDVPPPSAGSDASHPSTSSSQLDGLSVSLGRLGTRCEPEPSRLQAVFEALLTQFDRLNQATEDVYQLEQQLHSLQGRRSSRAPAGSSRGPSPGLRPALPSRLARASRGVDLATGPSRTPLRAKNKVHPSST

SEQ ID NO: 4 - DNA, 606 bp, synthetic construct
  source 1..606: mol_type = other DNA
ggggctgttattctccgctggcgctaccacgccttgcgtggagagctgtaccggccggcctgggagccccaggactacgagatggtggagttgttcctgcgcaggctgcgcctctggatgggcctcagcaaggtcaaggagttccgccacaaagtccgctttgaagggatggagccgctgccctctcgctcctccaggggctccaaggtatccccggatgtgcccccacccagcgctggctccgatgcctcgcacccctccacctcctccagccagctggatgggctgagcgtgagcctgggccggctggggacaaggtgtgagcctgagccctcccgcctccaagccgtgttcgaggccctgctcacccagtttgaccgactcaaccaggccacagaggacgtctaccagctggagcagcagctgcacagcctgcaaggccgcaggagcagccgggcgcccgccggatcttcccgtggcccatccccgggcctgcggccagcactgcccagccgccttgcccgggccagtcggggtgtggacctggccactggccccagcaggacaccccttcgggccaagaacaaggtccaccccagcagcact

SEQ ID NO: 5 - protein, 1256 aa, synthetic construct
MTAFGASLFVPPSHVRFVFPEPTADVNYIVMLTCAVCLVTYMVMAAILHKLDQLDASRGRAIPFCGQRGRFKYEILVKTGWGRGSGTTAHVGIMLYGVDSRSGHRHLDGDRAFHRNSLDIFRIATPHSLGSVWKIRVWHDNKGLSPAWFLQHVIVRDLQTARSAFFLVNDWLSVETEANGGLVEKEVLAASDAALLRFRRLLVAELQRGFFDKHIWLSIWDRPPRSRFTRIQRATCCVLLICLFLGANAVWYGAVGDSAYSTGHVSRLSPLSVDTVAVGLVSSVVVYPVYLAILFLFRMSRSKVAGSPSPTPAGQQVLDIDSCLDSSVLDSSFLTFSGLHAEQAFVGQMKSDLFLDDSKSLVCWPSGEGTLSWPDLLSDPSIVGSNLRQLARGQAGHGLGPEEDGFSLASPYSPAKSFSASDEDLIQQVLAEGVSSPAPTQDTHMETDLLSSLSSTPGEKTETLALQRLGELGPPSPGLNWEQPQAARLSRTGLVEGLRKRLLPAWCASLAHGLSLLLVAVAVAVSGWVGASFPPGVSVAWLLSSSASFLASFLGWEPLKVLLEALYFSLVAKRLHPDEDDTLVESPAVTPVSARVPRVRPPHGFALFLAKEEARKVKRLHGMLRSLLVYMLFLLVTLLASYGDASCHGHAYRLQSAIKQELHSRAFLAITRSEELWPWMAHVLLPYVHGNQSSPELGPPRLRQVRLQEALYPDPPGPRVHTCSAAGGFSTSDYDVGWESPHNGSGTWAYSAPDLLGAWSWGSCAVYDSGGYVQELGLSLEESRDRLRFLQLHNWLDNRSRAVFLELTRYSPAVGLHAAVTLRLEFPAAGRALAALSVRPFALRRLSAGLSLPLLTSVCLLLFAVHFAVAEARTWHREGRWRVLRLGAWARWLLVALTAATALVRLAQLGAADRQWTRFVRGRPRRFTSFDQVAQLSSAARGLAASLLFLLLVKAAQQLRFVRQWSVFGKTLCRALPELLGVTLGLVVLGVAYAQLAILLVSSCVDSLWSVAQALLVLCPGTGLSTLCPAESWHLSPLLCVGLWALRLWGALRLGAVILRWRYHALRGELYRPAWEPQDYEMVELFLRRLRLWMGLSKVKEFRHKVRFEGMEPLPSRSSRGSKVSPDVPPPSAGSDASHPSTSSSQLDGLSVSLGRLGTRCEPEPSRLQAVFEALLTQFDRLNQATEDVYQLEQQLHSLQGRRSSRAPAGSSRGPSPGLRPALPSRLARASRGVDLATGPSRTPLRAKNKVHPSST

SEQ ID NO: 6 - DNA, 3771 bp, synthetic construct
  source 1..3771: mol_type = other DNA
atgaccgccttcggcgccagcctcttcgtgcccccaagccatgtccgctttgtgtttcctgagccgacagcggatgtaaactacatcgtcatgctgacatgtgctgtgtgcctggtgacctacatggtcatggccgccatcctgcacaagctggaccagttggatgccagccggggccgcgccatccctttctgtgggcagcggggccgcttcaagtacgagatcctcgtcaagacaggctggggccggggctcaggtaccacggcccacgtgggcatcatgctgtatggggtggacagccggagcggccaccggcacctggacggcgacagagccttccaccgcaacagcctggacatcttccggatcgccaccccgcacagcctgggtagcgtgtggaagatccgagtgtggcacgacaacaaagggctcagccctgcctggttcctgcagcacgtcatcgtcagggacctgcagacggcacgcagcgccttcttcctggtcaatgactggctttcggtggagacggaggccaacgggggcctggtggagaaggaggtgctggccgcgagcgacgcagcccttttgcgcttccggcgcctgctggtggctgagctgcagcgtggcttctttgacaagcacatctggctctccatatgggaccggccgcctcgtagccgtttcactcgcatccagagggccacctgctgcgttctcctcatctgcctcttcctgggcgccaacgccgtgtggtacggggctgttggcgactctgcctacagcacggggcatgtgtccaggctgagcccgctgagcgtcgacacagtcgctgttggcctggtgtccagcgtggttgtctatcccgtctacctggccatcctttttctcttccggatgtcccggagcaaggtggctgggagcccgagccccacacctgccgggcagcaggtgctggacatcgacagctgcctggactcgtccgtgctggacagctccttcctcacgttctcaggcctccacgctgagcaggcctttgttggacagatgaagagtgacttgtttctggatgattctaagagtctggtgtgctggccctccggcgagggaacgctcagttggccggacctgctcagtgacccgtccattgtgggtagcaatctgcggcagctggcacggggccaggcgggccatgggctgggcccagaggaggacggcttctccctggccagcccctactcgcctgccaaatccttctcagcatcagatgaagacctgatccagcaggtccttgccgagggggtcagcagcccagcccctacccaagacacccacatggaaacggacctgctcagcagcctgtccagcactcctggggagaagacagagacgctggcgctgcagaggctgggggagctggggccacccagcccaggcctgaactgggaacagccccaggcagcgaggctgtccaggacaggactggtggagggtctgcggaagcgcctgctgccggcctggtgtgcctccctggcccacgggctcagcctgctcctggtggctgtggctgtggctgtctcagggtgggtgggtgcgagcttccccccgggcgtgagtgttgcgtggctcctgtccagcagcgccagcttcctggcctcattcctcggctgggagccactgaaggtcttgctggaagccctgtacttctcactggtggccaagcggctgcacccggatgaagatgacaccctggtagagagcccggctgtgacgcctgtgagcgcacgtgtgccccgcgtacggccaccccacggctttgcactcttcctggccaaggaagaagcccgcaaggtcaagaggctacatggcatgctgcggagcctcctggtgtacatgctttttctgctggtgaccctgctggccagctatggggatgcctcatgccatgggcacgcctaccgtctgcaaagcgccatcaagcaggagctgcacagccgggccttcctggccatcacgcggtctgaggagctctggccatggatggcccacgtgctgctgccctacgtccacgggaaccagtccagcccagagctggggcccccacggctgcggcaggtgcggctgcaggaagcactctacccagaccctcccggccccagggtccacacgtgctcggccgcaggaggcttcagcaccagcgattacgacgttggctgggagagtcctcacaatggctcggggacgtgggcctattcagcgccggatctgctgggggcatggtcctggggctcctgtgccgtgtatgacagcgggggctacgtgcaggagctgggcctgagcctggaggagagccgcgaccggctgcgcttcctgcagctgcacaactggctggacaacaggagccgcgctgtgttcctggagctcacgcgctacagcccggccgtggggctgcacgccgccgtcacgctgcgcctcgagttcccggcggccggccgcgccctggccgccctcagcgtccgcccctttgcgctgcgccgcctcagcgcgggcctctcgctgcctctgctcacctcggtgtgcctgctgctgttcgccgtgcacttcgccgtggccgaggcccgtacttggcacagggaagggcgctggcgcgtgctgcggctcggagcctgggcgcggtggctgctggtggcgctgacggcggccacggcactggtacgcctcgcccagctgggtgccgctgaccgccagtggacccgtttcgtgcgcggccgcccgcgccgcttcactagcttcgaccaggtggcgcagctgagctccgcagcccgtggcctggcggcctcgctgctcttcctgcttttggtcaaggctgcccagcagctacgcttcgtgcgccagtggtccgtctttggcaagacattatgccgagctctgccagagctcctgggggtcaccttgggcctggtggtgctcggggtagcctacgcccagctggccatcctgctcgtgtcttcctgtgtggactccctctggagcgtggcccaggccctgttggtgctgtgccctgggactgggctctctaccctgtgtcctgccgagtcctggcacctgtcacccctgctgtgtgtggggctctgggcactgcggctgtggggcgccctacggctgggggctgttattctccgctggcgctaccacgccttgcgtggagagctgtaccggccggcctgggagccccaggactacgagatggtggagttgttcctgcgcaggctgcgcctctggatgggcctcagcaaggtcaaggagttccgccacaaagtccgctttgaagggatggagccgctgccctctcgctcctccaggggctccaaggtatccccggatgtgcccccacccagcgctggctccgatgcctcgcacccctccacctcctccagccagctggatgggctgagcgtgagcctgggccggctggggacaaggtgtgagcctgagccctcccgcctccaagccgtgttcgaggccctgctcacccagtttgaccgactcaaccaggccacagaggacgtctaccagctggagcagcagctgcacagcctgcaaggccgcaggagcagccgggcgcccgccggatcttcccgtggcccatccccgggcctgcggccagcactgcccagccgccttgcccgggccagtcggggtgtggacctggccactggccccagcaggacaccccttcgggccaagaacaaggtccaccccagcagcacttaa

SEQ ID NO: 7 - protein, 203 aa, synthetic construct
MGAVILRWRYHALRGELYRPAWEPQDYEMVELFLRRLRLWMGLSKVKEFRHKVRFEGMEPLPSRSSRGSKVSPDVPPPSAGSDASHPSTSSSQLDGLSVSLGRLGTRCEPEPSRLQAVFEALLTQFDRLNQATEDVYQLEQQLHSLQGRRSSRAPAGSSRGPSPGLRPALPSRLARASRGVDLATGPSRTPLRAKNKVHPSST

SEQ ID NO: 8 - DNA, 612 bp, synthetic construct
  source 1..612: mol_type = other DNA
atgggggctgttattctccgctggcgctaccacgccttgcgtggagagctgtaccggccggcctgggagccccaggactacgagatggtggagttgttcctgcgcaggctgcgcctctggatgggcctcagcaaggtcaaggagttccgccacaaagtccgctttgaagggatggagccgctgccctctcgctcctccaggggctccaaggtatccccggatgtgcccccacccagcgctggctccgatgcctcgcacccctccacctcctccagccagctggatgggctgagcgtgagcctgggccggctggggacaaggtgtgagcctgagccctcccgcctccaagccgtgttcgaggccctgctcacccagtttgaccgactcaaccaggccacagaggacgtctaccagctggagcagcagctgcacagcctgcaaggccgcaggagcagccgggcgcccgccggatcttcccgtggcccatccccgggcctgcggccagcactgcccagccgccttgcccgggccagtcggggtgtggacctggccactggccccagcaggacaccccttcgggccaagaacaaggtccaccccagcagcacttaa

SEQ ID NO: 9 - protein, 1768 aa, synthetic construct
MPPAAPARLALALGLGLWLGALAGGPGRGCGPCEPPCLCGPAPGAACRVNCSGRGLRTLGPALRIPADATALDVSHNLLRALDVGLLANLSALAELDISNNKISTLEEGIFANLFNLSEINLSGNPFECDCGLAWLPRWAEEQQVRVVQPEAATCAGPGSLAGQPLLGIPLLDSGCGEEYVACLPDNSSGTVAAVSFSAAHEGLLQPEACSAFCFSTGQGLAALSEQGWCLCGAAQPSSASFACLSLCSGPPPPPAPTCRGPTLLQHVFPASPGATLVGPHGPLASGQLAAFHIAAPLPVTATRWDFGDGSAEVDAAGPAASHRYVLPGRYHVTAVLALGAGSALLGTDVQVEAAPAALELVCPSSVQSDESLDLSIQNRGGSGLEAAYSIVALGEEPARAVHPLCPSDTEIFPGNGHCYRLVVEKAAWLQAQEQCQAWAGAALAMVDSPAVQRFLVSRVTRSLDVWIGFSTVQGVEVGPAPQGEAFSLESCQNWLPGEPHPATAEHCVRLGPTGWCNTDLCSAPHSYVCELQPGGPVQDAENLLVGAPSGDLQGPLTPLAQQDGLSAPHEPVEVMVFPGLRLSREAFLTTAEFGTQELRRPAQLRLQVYRLLSTAGTPENGSEPESRSPDNRTQLAPACMPGGRWCPGANICLPLDASCHPQACANGCTSGPGLPGAPYALWREFLFSVPAGPPAQYSVTLHGQDVLMLPGDLVGLQHDAGPGALLHCSPAPGHPGPRAPYLSANASSWLPHLPAQLEGTWACPACALRLLAATEQLTVLLGLRPNPGLRLPGRYEVRAEVGNGVSRHNLSCSFDVVSPVAGLRVIYPAPRDGRLYVPTNGSALVLQVDSGANATATARWPGGSVSARFENVCPALVATFVPGCPWETNDTLFSVVALPWLSEGEHVVDVVVENSASRANLSLRVTAEEPICGLRATPSPEARVLQGVLVRYSPVVEAGSDMVFRWTINDKQSLTFQNVVFNVIYQSAAVFKLSLTASNHVSNVTVNYNVTVERMNRMQGLQVSTVPAVLSPNATLALTAGVLVDSAVEVAFLWTFGDGEQALHQFQPPYNESFPVPDPSVAQVLVEHNVMHTYAAPGEYLLTVLASNAFENLTQQVPVSVRASLPSVAVGVSDGVLVAGRPVTFYPHPLPSPGGVLYTWDFGDGSPVLTQSQPAANHTYASRGTYHVRLEVNNTVSGAAAQADVRVFEELRGLSVDMSLAVEQGAPVVVSAAVQTGDNITWTFDMGDGTVLSGPEATVEHVYLRAQNCTVTVGAASPAGHLARSLHVLVFVLEVLRVEPAACIPTQPDARLTAYVTGNPAHYLFDWTFGDGSSNTTVRGCPTVTHNFTRSGTFPLALVLSSRVNRAHYFTSICVEPEVGNVTLQPERQFVQLGDEAWLVACAWPPFPYRYTWDFGTEEAAPTRARGPEVTFIYRDPGSYLVTVTASNNISAANDSALVEVQEPVLVTSIKVNGSLGLELQQPYLFSAVGRGRPASYLWDLGDGGWLEGPEVTHAYNSTGDFTVRVAGWNEVSRSEAWLNVTVKRRVRGLVVNASRTVVPLNGSVSFSTSLEAGSDVRYSWVLCDRCTPIPGGPTISYTFRSVGTFNIIVTAENEVGSAQDSIFVYVLQLIEGLQVVGGGRYFPTNHTVQLQAVVRDGTNVSYSWTAWRDGPGPGRQRQRLLAHRARGRHLPCAAAGHQHAGQRLGRLHHGLRGACGVADGGRLPEPSCRQHKRHPQCRAGWWQWCRIHLVLGGGAELGDLRAIYHP

SEQ ID NO: 10 - DNA, 12910 bp, synthetic construct
  source 1..12910: mol_type = other DNA
atgccgcccgccgcgcccgcccgcctggcgctggccctgggcctgggcctgtggctcggggcgctggcggggggccccgggcgcggctgcgggccctgcgagcccccctgcctctgcggcccagcgcccggcgccgcctgccgcgtcaactgctcgggccgcgggctgcggacgctcggtcccgcgctgcgcatccccgcggacgccacagcgctagacgtctcccacaacctgctccgggcgctggacgttgggctcctggcgaacctctcggcgctggcagagctggatataagcaacaacaagatttctacgttagaagaaggaatatttgctaatttatttaatttaagtgaaataaacctgagtgggaacccgtttgagtgtgactgtggcctggcgtggctgccgcgatgggcggaggagcagcaggtgcgggtggtgcagcccgaggcagccacgtgtgctgggcctggctccctggctggccagcctctgcttggcatccccttgctggacagtggctgtggtgaggagtatgtcgcctgcctccctgacaacagctcaggcaccgtggcagcagtgtccttttcagctgcccacgaaggcctgcttcagccagaggcctgcagcgccttctgcttctccaccggccagggcctcgcagccctctcggagcagggctggtgcctgtgtggggcggcccagccctccagtgcctcctttgcctgcctgtccctctgctccggccccccgccacctcctgcccccacctgtaggggccccaccctcctccagcacgtcttccctgcctccccaggggccaccctggtggggccccacggacctctggcctctggccagctagcagccttccacatcgctgccccgctccctgtcactgccacacgctgggacttcggagacggctccgccgaggtggatgccgctgggccggctgcctcgcatcgctatgtgctgcctgggcgctatcacgtgacggccgtgctggccctgggggccggctcagccctgctggggacagacgtgcaggtggaagcggcacctgccgccctggagctcgtgtgcccgtcctcggtgcagagtgacgagagcctcgacctcagcatccagaaccgcggtggttcaggcctggaggccgcctacagcatcgtggccctgggcgaggagccggcccgagcggtgcacccgctctgcccctcggacacggagatcttccctggcaacgggcactgctaccgcctggtggtggagaaggcggcctggctgcaggcgcaggagcagtgtcaggcctgggccggggccgccctggcaatggtggacagtcccgccgtgcagcgcttcctggtctcccgggtcaccaggagcctagacgtgtggatcggcttctcgactgtgcagggggtggaggtgggcccagcgccgcagggcgaggccttcagcctggagagctgccagaactggctgcccggggagccacacccagccacagccgagcactgcgtccggctcgggcccaccgggtggtgtaacaccgacctgtgctcagcgccgcacagctacgtctgcgagctgcagcccggaggcccagtgcaggatgccgagaacctcctcgtgggagcgcccagtggggacctgcagggacccctgacgcctctggcacagcaggacggcctctcagccccgcacgagcccgtggaggtcatggtattcccgggcctgcgtctgagccgtgaagccttcctcaccacggccgaatttgggacccaggagctccggcggcccgcccagctgcggctgcaggtgtaccggctcctcagcacagcagggaccccggagaacggcagcgagcctgagagcaggtccccggacaacaggacccagctggcccccgcgtgcatgccagggggacgctggtgccctggagccaacatctgcttgccgctggacgcctcctgccacccccaggcctgcgccaatggctgcacgtcagggccagggctacccggggccccctatgcgctatggagagagttcctcttctccgttcccgcggggccccccgcgcagtactcggtcaccctccacggccaggatgtcctcatgctccctggtgacctcgttggcttgcagcacgacgctggccctggcgccctcctgcactgctcgccggctcccggccaccctggtccccgggccccgtacctctccgccaacgcctcgtcatggctgccccacttgccagcccagctggagggcacttgggcctgccctgcctgtgccctgcggctgcttgcagccacggaacagctcaccgtgctgctgggcttgaggcccaaccctggactgcggctgcctgggcgctatgaggtccgggcagaggtgggcaatggcgtgtccaggcacaacctctcctgcagctttgacgtggtctccccagtggctgggctgcgggtcatctaccctgccccccgcgacggccgcctctacgtgcccaccaacggctcagccttggtgctccaggtggactctggtgccaacgccacggccacggctcgctggcctgggggcagtgtcagcgcccgctttgagaatgtctgccctgccctggtggccaccttcgtgcccggctgcccctgggagaccaacgataccctgttctcagtggtagcactgccgtggctcagtgagggggagcacgtggtggacgtggtggtggaaaacagcgccagccgggccaacctcagcctgcgggtgacggcggaggagcccatctgtggcctccgcgccacgcccagccccgaggcccgtgtactgcagggagtcctagtgaggtacagccccgtggtggaggccggctcggacatggtcttccggtggaccatcaacgacaagcagtccctgaccttccagaacgtggtcttcaatgtcatttatcagagcgcggcggtcttcaagctctcactgacggcctccaaccacgtgagcaacgtcaccgtgaactacaacgtaaccgtggagcggatgaacaggatgcagggtctgcaggtctccacagtgccggccgtgctgtcccccaatgccacgctagcactgacggcgggcgtgctggtggactcggccgtggaggtggccttcctgtggacctttggggatggggagcaggccctccaccagttccagcctccgtacaacgagtccttcccggttccagacccctcggtggcccaggtgctggtggagcacaatgtcatgcacacctacgctgccccaggtgagtacctcctgaccgtgctggcatctaatgccttcgagaacctgacgcagcaggtgcctgtgagcgtgcgcgcctccctgccctccgtggctgtgggtgtgagtgacggcgtcctggtggccggccggcccgtcaccttctacccgcacccgctgccctcgcctgggggtgttctttacacgtgggacttcggggacggctcccctgtcctgacccagagccagccggctgccaaccacacctatgcctcgaggggcacctaccacgtgcgcctggaggtcaacaacacggtgagcggtgcggcggcccaggcggatgtgcgcgtctttgaggagctccgcggactcagcgtggacatgagcctggccgtggagcagggcgcccccgtggtggtcagcgccgcggtgcagacgggcgacaacatcacgtggaccttcgacatgggggacggcaccgtgctgtcgggcccggaggcaacagtggagcatgtgtacctgcgggcacagaactgcacagtgaccgtgggtgcggccagccccgccggccacctggcccggagcctgcacgtgctggtcttcgtcctggaggtgctgcgcgttgaacccgccgcctgcatccccacgcagcctgacgcgcggctcacggcctacgtcaccgggaacccggcccactacctcttcgactggaccttcggggatggctcctccaacacgaccgtgcgggggtgcccgacggtgacacacaacttcacgcggagcggcacgttccccctggcgctggtgctgtccagccgcgtgaacagggcgcattacttcaccagcatctgcgtggagccagaggtgggcaacgtcaccctgcagccagagaggcagtttgtgcagctcggggacgaggcctggctggtggcatgtgcctggcccccgttcccctaccgctacacctgggactttggcaccgaggaagccgcccccacccgtgccaggggccctgaggtgacgttcatctaccgagacccaggctcctatcttgtgacagtcaccgcgtccaacaacatctctgctgccaatgactcagccctggtggaggtgcaggagcccgtgctggtcaccagcatcaaggtcaatggctcccttgggctggagctgcagcagccgtacctgttctctgctgtgggccgtgggcgccccgccagctacctgtgggatctgggggacggtgggtggctcgagggtccggaggtcacccacgcttacaacagcacaggtgacttcaccgttagggtggccggctggaatgaggtgagccgcagcgaggcctggctcaatgtgacggtgaagcggcgcgtgcgggggctcgtcgtcaatgcaagccgcacggtggtgcccctgaatgggagcgtgagcttcagcacgtcgctggaggccggcagtgatgtgcgctattcctgggtgctctgtgaccgctgcacgcccatccctgggggtcctaccatctcttacaccttccgctccgtgggcaccttcaatatcatcgtcacggctgagaacgaggtgggctccgcccaggacagcatcttcgtctatgtcctgcagctcatagaggggctgcaggtggtgggcggtggccgctacttccccaccaaccacacggtacagctgcaggccgtggttagggatggcaccaacgtctcctacagctggactgcctggagggacgggcccggccctggccggcagcggcaaaggcttctcgctcaccgtgctcgaggccggcacctaccatgtgcagctgcgggccaccaacatgctgggcagcgcctgggccgactgcaccatggacttcgtggagcctgtggggtggctgatggtggccgcctccccgaacccagctgccgtcaacacaagcgtcaccctcagtgccgagctggctggtggcagtggtgtcgtatacacttggtccttggaggaggggctgagctgggagacctccgagccatttaccacccatagcttccccacacccggcctgcacttggtcaccatgacggcagggaacccgctgggctcagccaacgccaccgtggaagtggatgtgcaggtgcctgtgagtggcctcagcatcagggccagcgagcccggaggcagcttcgtggcggccgggtcctctgtgcccttttgggggcagctggccacgggcaccaatgtgagctggtgctgggctgtgcccggcggcagcagcaagcgtggccctcatgtcaccatggtcttcccggatgctggcaccttctccatccggctcaatgcctccaacgcagtcagctgggtctcagccacgtacaacctcacggcggaggagcccatcgtgggcctggtgctgtgggccagcagcaaggtggtggcgcccgggcagctggtccattttcagatcctgctggctgccggctcagctgtcaccttccgcctgcaggtcggcggggccaaccccgaggtgctccccgggccccgtttctcccacagcttcccccgcgtcggagaccacgtggtgagcgtgcggggcaaaaaccacgtgagctgggcccaggcgcaggtgcgcatcgtggtgctggaggccgtgagtgggctgcaggtgcccaactgctgcgagcctggcatcgccacgggcactgagaggaacttcacagcccgcgtgcagcgcggctctcgggtcgcctacgcctggtacttctcgctgcagaaggtccagggcgactcgctggtcatcctgtcgggccgcgacgtcacctacacgcccgtggccgcggggctgttggagatccaggtgcgcgccttcaacgccctgggcagtgagaaccgcacgctggtgctggaggttcaggacgccgtccagtatgtggccctgcagagcggcccctgcttcaccaaccgctcggcgcagtttgaggccgccaccagccccagcccccggcgtgtggcctaccactgggactttggggatgggtcgccagggcaggacacagatgagcccagggccgagcactcctacctgaggcctggggactaccgcgtgcaggtgaacgcctccaacctggtgagcttcttcgtggcgcaggccacggtgaccgtccaggtgctggcctgccgggagccggaggtggacgtggtcctgcccctgcaggtgctgatgcggcgatcacagcgcaactacttggaggcccacgttgacctgcgcgactgcgtcacctaccagactgagtaccgctgggaggtgtatcgcaccgccagctgccagcggccggggcgcccagcgcgtgtggccctgcccggcgtggacgtgagccggcctcggctggtgctgccgcggctggcgctgcctgtggggcactactgctttgtgtttgtcgtgtcatttggggacacgccactgacacagagcatccaggccaatgtgacggtggcccccgagcgcctggtgcccatcattgagggtggctcataccgcgtgtggtcagacacacgggacctggtgctggatgggagcgagtcctacgaccccaacctggaggacggcgaccagacgccgctcagtttccactgggcctgtgtggcttcgacacagagggaggctggcgggtgtgcgctgaactttgggccccgcgggagcagcacggtcaccattccacgggagcggctggcggctggcgtggagtacaccttcagcctgaccgtgtggaaggccggccgcaaggaggaggccaccaaccagacggtgctgatccggagtggccgggtgcccattgtgtccttggagtgtgtgtcctgcaaggcacaggccgtgtacgaagtgagccgcagctcctacgtgtacttggagggccgctgcctcaattgcagcagcggctccaagcgagggcggtgggctgcacgtacgttcagcaacaagacgctggtgctggatgagaccaccacatccacgggcagtgcaggcatgcgactggtgctgcggcggggcgtgctgcgggacggcgagggatacaccttcacgctcacggtgctgggccgctctggcgaggaggagggctgcgcctccatccgcctgtcccccaaccgcccgccgctggggggctcttgccgcctcttcccactgggcgctgtgcacgccctcaccaccaaggtgcacttcgaatgcacgggctggcatgacgcggaggatgctggcgccccgctggtgtacgccctgctgctgcggcgctgtcgccagggccactgcgaggagttctgtgtctacaagggcagcctctccagctacggagccgtgctgcccccgggtttcaggccacacttcgaggtgggcctggccgtggtggtgcaggaccagctgggagccgctgtggtcgccctcaacaggtctttggccatcaccctcccagagcccaacggcagcgcaacggggctcacagtctggctgcacgggctcaccgctagtgtgctcccagggctgctgcggcaggccgatccccagcacgtcatcgagtactcgttggccctggtcaccgtgctgaacgagtacgagcgggccctggacgtggcggcagagcccaagcacgagcggcagcaccgagcccagatacgcaagaacatcacggagactctggtgtccctgagggtccacactgtggatgacatccagcagatcgctgctgcgctggcccagtgcatggggcccagcagggagctcgtatgccgctcgtgcctgaagcagacgctgcacaagctggaggccatgatgctcatcctgcaggcagagaccaccgcgggcaccgtgacgcccaccgccatcggagacagcatcctcaacatcacaggagacctcatccacctggccagctcggacgtgcgggcaccacagccctcagagctgggagccgagtcaccatctcggatggtggcgtcccaggcctacaacctgacctctgccctcatgcgcatcctcatgcgctcccgcgtgctcaacgaggagcccctgacgctggcgggcgaggagatcgtggcccagggcaagcgctcggacccgcggagcctgctgtgctatggcggcgccccagggcctggctgccacttctccatccccgaggctttcagcggggccctggccaacctcagtgacgtggtgcagctcatctttctggtggactccaatccctttccctttggctatatcagcaactacaccgtctccaccaaggtggcctcgatggcattccagacacaggccggcgcccagatccccatcgagcggctggcctcagagcgcgccatcaccgtgaaggtgcccaacaactcggactgggctgcccggggccaccgcagctccgccaactccgccaactccgttgtggtccagccccaggcctccgtcggtgctgtggtcaccctggacagcagcaaccctgcggccgggctgcatctgcagctcaactatacgctgctggacggccactacctgtctgaggaacctgagccctacctggcagtctacctacactcggagccccggcccaatgagcacaactgctcggctagcaggaggatccgcccagagtcactccagggtgctgaccaccggccctacaccttcttcatttccccggggagcagagacccagcggggagttaccatctgaacctctccagccacttccgctggtcggcgctgcaggtgtccgtgggcctgtacacgtccctgtgccagtacttcagcgaggaggacatggtgtggcggacagaggggctgctgcccctggaggagacctcgccccgccaggccgtctgcctcacccgccacctcaccgccttcggcgccagcctcttcgtgcccccaagccatgtccgctttgtgtttcctgagccgacagcggatgtaaactacatcgtcatgctgacatgtgctgtgtgcctggtgacctacatggtcatggccgccatcctgcacaagctggaccagttggatgccagccggggccgcgccatccctttctgtgggcagcggggccgcttcaagtacgagatcctcgtcaagacaggctggggccggggctcaggtaccacggcccacgtgggcatcatgctgtatggggtggacagccggagcggccaccggcacctggacggcgacagagccttccaccgcaacagcctggacatcttccggatcgccaccccgcacagcctgggtagcgtgtggaagatccgagtgtggcacgacaacaaagggctcagccctgcctggttcctgcagcacgtcatcgtcagggacctgcagacggcacgcagcgccttcttcctggtcaatgactggctttcggtggagacggaggccaacgggggcctggtggagaaggaggtgctggccgcgagcgacgcagcccttttgcgcttccggcgcctgctggtggctgagctgcagcgtggcttctttgacaagcacatctggctctccatatgggaccggccgcctcgtagccgtttcactcgcatccagagggccacctgctgcgttctcctcatctgcctcttcctgggcgccaacgccgtgtggtacggggctgttggcgactctgcctacagcacggggcatgtgtccaggctgagcccgctgagcgtcgacacagtcgctgttggcctggtgtccagcgtggttgtctatcccgtctacctggccatcctttttctcttccggatgtcccggagcaaggtggctgggagcccgagccccacacctgccgggcagcaggtgctggacatcgacagctgcctggactcgtccgtgctggacagctccttcctcacgttctcaggcctccacgctgagcaggcctttgttggacagatgaagagtgacttgtttctggatgattctaagagtctggtgtgctggccctccggcgagggaacgctcagttggccggacctgctcagtgacccgtccattgtgggtagcaatctgcggcagctggcacggggccaggcgggccatgggctgggcccagaggaggacggcttctccctggccagcccctactcgcctgccaaatccttctcagcatcagatgaagacctgatccagcaggtccttgccgagggggtcagcagcccagcccctacccaagacacccacatggaaacggacctgctcagcagcctgtccagcactcctggggagaagacagagacgctggcgctgcagaggctgggggagctggggccacccagcccaggcctgaactgggaacagccccaggcagcgaggctgtccaggacaggactggtggagggtctgcggaagcgcctgctgccggcctggtgtgcctccctggcccacgggctcagcctgctcctggtggctgtggctgtggctgtctcagggtgggtgggtgcgagcttccccccgggcgtgagtgttgcgtggctcctgtccagcagcgccagcttcctggcctcattcctcggctgggagccactgaaggtcttgctggaagccctgtacttctcactggtggccaagcggctgcacccggatgaagatgacaccctggtagagagcccggctgtgacgcctgtgagcgcacgtgtgccccgcgtacggccaccccacggctttgcactcttcctggccaaggaagaagcccgcaaggtcaagaggctacatggcatgctgcggagcctcctggtgtacatgctttttctgctggtgaccctgctggccagctatggggatgcctcatgccatgggcacgcctaccgtctgcaaagcgccatcaagcaggagctgcacagccgggccttcctggccatcacgcggtctgaggagctctggccatggatggcccacgtgctgctgccctacgtccacgggaaccagtccagcccagagctggggcccccacggctgcggcaggtgcggctgcaggaagcactctacccagaccctcccggccccagggtccacacgtgctcggccgcaggaggcttcagcaccagcgattacgacgttggctgggagagtcctcacaatggctcggggacgtgggcctattcagcgccggatctgctgggggcatggtcctggggctcctgtgccgtgtatgacagcgggggctacgtgcaggagctgggcctgagcctggaggagagccgcgaccggctgcgcttcctgcagctgcacaactggctggacaacaggagccgcgctgtgttcctggagctcacgcgctacagcccggccgtggggctgcacgccgccgtcacgctgcgcctcgagttcccggcggccggccgcgccctggccgccctcagcgtccgcccctttgcgctgcgccgcctcagcgcgggcctctcgctgcctctgctcacctcggtgtgcctgctgctgttcgccgtgcacttcgccgtggccgaggcccgtacttggcacagggaagggcgctggcgcgtgctgcggctcggagcctgggcgcggtggctgctggtggcgctgacggcggccacggcactggtacgcctcgcccagctgggtgccgctgaccgccagtggacccgtttcgtgcgcggccgcccgcgccgcttcactagcttcgaccaggtggcgcagctgagctccgcagcccgtggcctggcggcctcgctgctcttcctgcttttggtcaaggctgcccagcagctacgcttcgtgcgccagtggtccgtctttggcaagacattatgccgagctctgccagagctcctgggggtcaccttgggcctggtggtgctcggggtagcctacgcccagctggccatcctgctcgtgtcttcctgtgtggactccctctggagcgtggcccaggccctgttggtgctgtgccctgggactgggctctctaccctgtgtcctgccgagtcctggcacctgtcacccctgctgtgtgtggggctctgggcactgcggctgtggggcgccctacggctgggggctgttattctccgctggcgctaccacgccttgcgtggagagctgtaccggccggcctgggagccccaggactacgagatggtggagttgttcctgcgcaggctgcgcctctggatgggcctcagcaaggtcaaggagttccgccacaaagtccgctttgaagggatggagccgctgccctctcgctcctccaggggctccaaggtatccccggatgtgcccccacccagcgctggctccgatgcctcgcacccctccacctcctccagccagctggatgggctgagcgtgagcctgggccggctggggacaaggtgtgagcctgagccctcccgcctccaagccgtgttcgaggccctgctcacccagtttgaccgactcaaccaggccacagaggacgtctaccagctggagcagcagctgcacagcctgcaaggccgcaggagcagccgggcgcccgccggatcttcccgtggcccatccccgggcctgcggccagcactgcccagccgccttgcccgggccagtcggggtgtggacctggccactggccccagcaggacaccccttcgggccaagaacaaggtccaccccagcagcacttaa

SEQ ID NO: 11 - protein, 1030 aa, synthetic construct
MTAFGASLFVPPSHVRFVFPEPTADVNYIVMLTCAVCLVTYMVMAAILHKLDQLDASRGRAIPFCGQRGRFKYEILVKTGWGRGSGTTAHVGIMLYGVDSRSGHRHLDGDRAFHRNSLDIFRIATPHSLGSVWKIRVWHDNKGLSPAWFLQHVIVRDLQTARSAFFLVNDWLSVETEANGGLVEKEVLAASDAALLRFRRLLVAELQRGFFDKHIWLSIWDRPPRSRFTRIQRATCCVLLICLFLGANAVWYGAVGDSAYSTGHVSRLSPLSVDTVAVGLVSSVVVYPVYLAILFLFRMSRSKVAGSPSPTPAGQQVLDIDSCLDSSVLDSSFLTFSGLHAEQAFVGQMKSDLFLDDSKSLVCWPSGEGTLSWPDLLSDPSIVGSNLRQLARGQAGHGLGPEEDGFSLASPYSPAKSFSASDEDLIQQVLAEGVSSPAPTQDTHMETDLLSSLSSTPGEKTETLALQRLGELGPPSPGLNWEQPQAARLSRTGLVEGLRKRLLPAWCASLAHGLSLLLVAVAVAVSGWVGASFPPGVSVAWLLSSSASFLASFLGWEPLKVLLEALYFSLVAKRLHPDEDDTLVESPAVTPVSARVPRVRPPHGFALFLAKEEARKVKRLHGMLRSLLVYMLFLLVTLLASYGDASCHGHAYRLQSAIKQELHSRAFLAITRSEELWPWMAHVLLPYVHGNQSSPELGPPRLRQVRLQEALYPDPPGPRVHTCSAAGGFSTSDYDVGWESPHNGSGTWAYSAPDLLGAWSWGSCAVYDSGGYVQELGLSLEESRDRLRFLQLHNWLDNRSRAVFLELTRYSPAVGLHAAVTLRLEFPAAGRALAALSVRPFALRRLSAGLSLPLLTSVCLLLFAVHFAVAEARTWHREGRWRVLRLGAWARWLLVALTAATALVRLAQLGAADRQWTRFVRGRPRRFTSFDQVAQLSSAARGLAASLLFLLLVKAAQQLRFVRQWSVFGKTLCRALPELLGVTLGLVVLGVAYAQLAILLVSSCVDSLWSVAQALLVLCPGTGLSTLCPA

SEQ ID NO: 12 - DNA, 3093 bp, synthetic construct
  source 1..3093: mol_type = other DNA
atgaccgccttcggcgccagcctcttcgtgcccccaagccatgtccgctttgtgtttcctgagccgacagcggatgtaaactacatcgtcatgctgacatgtgctgtgtgcctggtgacctacatggtcatggccgccatcctgcacaagctggaccagttggatgccagccggggccgcgccatccctttctgtgggcagcggggccgcttcaagtacgagatcctcgtcaagacaggctggggccggggctcaggtaccacggcccacgtgggcatcatgctgtatggggtggacagccggagcggccaccggcacctggacggcgacagagccttccaccgcaacagcctggacatcttccggatcgccaccccgcacagcctgggtagcgtgtggaagatccgagtgtggcacgacaacaaagggctcagccctgcctggttcctgcagcacgtcatcgtcagggacctgcagacggcacgcagcgccttcttcctggtcaatgactggctttcggtggagacggaggccaacgggggcctggtggagaaggaggtgctggccgcgagcgacgcagcccttttgcgcttccggcgcctgctggtggctgagctgcagcgtggcttctttgacaagcacatctggctctccatatgggaccggccgcctcgtagccgtttcactcgcatccagagggccacctgctgcgttctcctcatctgcctcttcctgggcgccaacgccgtgtggtacggggctgttggcgactctgcctacagcacggggcatgtgtccaggctgagcccgctgagcgtcgacacagtcgctgttggcctggtgtccagcgtggttgtctatcccgtctacctggccatcctttttctcttccggatgtcccggagcaaggtggctgggagcccgagccccacacctgccgggcagcaggtgctggacatcgacagctgcctggactcgtccgtgctggacagctccttcctcacgttctcaggcctccacgctgagcaggcctttgttggacagatgaagagtgacttgtttctggatgattctaagagtctggtgtgctggccctccggcgagggaacgctcagttggccggacctgctcagtgacccgtccattgtgggtagcaatctgcggcagctggcacggggccaggcgggccatgggctgggcccagaggaggacggcttctccctggccagcccctactcgcctgccaaatccttctcagcatcagatgaagacctgatccagcaggtccttgccgagggggtcagcagcccagcccctacccaagacacccacatggaaacggacctgctcagcagcctgtccagcactcctggggagaagacagagacgctggcgctgcagaggctgggggagctggggccacccagcccaggcctgaactgggaacagccccaggcagcgaggctgtccaggacaggactggtggagggtctgcggaagcgcctgctgccggcctggtgtgcctccctggcccacgggctcagcctgctcctggtggctgtggctgtggctgtctcagggtgggtgggtgcgagcttccccccgggcgtgagtgttgcgtggctcctgtccagcagcgccagcttcctggcctcattcctcggctgggagccactgaaggtcttgctggaagccctgtacttctcactggtggccaagcggctgcacccggatgaagatgacaccctggtagagagcccggctgtgacgcctgtgagcgcacgtgtgccccgcgtacggccaccccacggctttgcactcttcctggccaaggaagaagcccgcaaggtcaagaggctacatggcatgctgcggagcctcctggtgtacatgctttttctgctggtgaccctgctggccagctatggggatgcctcatgccatgggcacgcctaccgtctgcaaagcgccatcaagcaggagctgcacagccgggccttcctggccatcacgcggtctgaggagctctggccatggatggcccacgtgctgctgccctacgtccacgggaaccagtccagcccagagctggggcccccacggctgcggcaggtgcggctgcaggaagcactctacccagaccctcccggccccagggtccacacgtgctcggccgcaggaggcttcagcaccagcgattacgacgttggctgggagagtcctcacaatggctcggggacgtgggcctattcagcgccggatctgctgggggcatggtcctggggctcctgtgccgtgtatgacagcgggggctacgtgcaggagctgggcctgagcctggaggagagccgcgaccggctgcgcttcctgcagctgcacaactggctggacaacaggagccgcgctgtgttcctggagctcacgcgctacagcccggccgtggggctgcacgccgccgtcacgctgcgcctcgagttcccggcggccggccgcgccctggccgccctcagcgtccgcccctttgcgctgcgccgcctcagcgcgggcctctcgctgcctctgctcacctcggtgtgcctgctgctgttcgccgtgcacttcgccgtggccgaggcccgtacttggcacagggaagggcgctggcgcgtgctgcggctcggagcctgggcgcggtggctgctggtggcgctgacggcggccacggcactggtacgcctcgcccagctgggtgccgctgaccgccagtggacccgtttcgtgcgcggccgcccgcgccgcttcactagcttcgaccaggtggcgcagctgagctccgcagcccgtggcctggcggcctcgctgctcttcctgcttttggtcaaggctgcccagcagctacgcttcgtgcgccagtggtccgtctttggcaagacattatgccgagctctgccagagctcctgggggtcaccttgggcctggtggtgctcggggtagcctacgcccagctggccatcctgctcgtgtcttcctgtgtggactccctctggagcgtggcccaggccctgttggtgctgtgccctgggactgggctctctaccctgtgtcctgcctaa

SEQ ID NO: 13 - protein, 1004 aa, synthetic construct
MYIVMLTCAVCLVTYMVMAAILHKLDQLDASRGRAIPFCGQRGRFKYEILVKTGWGRGSGTTAHVGIMLYGVDSRSGHRHLDGDRAFHRNSLDIFRIATPHSLGSVWKIRVWHDNKGLSPAWFLQHVIVRDLQTARSAFFLVNDWLSVETEANGGLVEKEVLAASDAALLRFRRLLVAELQRGFFDKHIWLSIWDRPPRSRFTRIQRATCCVLLICLFLGANAVWYGAVGDSAYSTGHVSRLSPLSVDTVAVGLVSSVVVYPVYLAILFLFRMSRSKVAGSPSPTPAGQQVLDIDSCLDSSVLDSSFLTFSGLHAEQAFVGQMKSDLFLDDSKSLVCWPSGEGTLSWPDLLSDPSIVGSNLRQLARGQAGHGLGPEEDGFSLASPYSPAKSFSASDEDLIQQVLAEGVSSPAPTQDTHMETDLLSSLSSTPGEKTETLALQRLGELGPPSPGLNWEQPQAARLSRTGLVEGLRKRLLPAWCASLAHGLSLLLVAVAVAVSGWVGASFPPGVSVAWLLSSSASFLASFLGWEPLKVLLEALYFSLVAKRLHPDEDDTLVESPAVTPVSARVPRVRPPHGFALFLAKEEARKVKRLHGMLRSLLVYMLFLLVTLLASYGDASCHGHAYRLQSAIKQELHSRAFLAITRSEELWPWMAHVLLPYVHGNQSSPELGPPRLRQVRLQEALYPDPPGPRVHTCSAAGGFSTSDYDVGWESPHNGSGTWAYSAPDLLGAWSWGSCAVYDSGGYVQELGLSLEESRDRLRFLQLHNWLDNRSRAVFLELTRYSPAVGLHAAVTLRLEFPAAGRALAALSVRPFALRRLSAGLSLPLLTSVCLLLFAVHFAVAEARTWHREGRWRVLRLGAWARWLLVALTAATALVRLAQLGAADRQWTRFVRGRPRRFTSFDQVAQLSSAARGLAASLLFLLLVKAAQQLRFVRQWSVFGKTLCRALPELLGVTLGLVVLGVAYAQLAILLVSSCVDSLWSVAQALLVLCPGTGLSTLCPA

SEQ ID NO: 14 - DNA, 3015 bp, synthetic construct
  source 1..3015: mol_type = other DNA
atgtacatcgtcatgctgacatgtgctgtgtgcctggtgacctacatggtcatggccgccatcctgcacaagctggaccagttggatgccagccggggccgcgccatccctttctgtgggcagcggggccgcttcaagtacgagatcctcgtcaagacaggctggggccggggctcaggtaccacggcccacgtgggcatcatgctgtatggggtggacagccggagcggccaccggcacctggacggcgacagagccttccaccgcaacagcctggacatcttccggatcgccaccccgcacagcctgggtagcgtgtggaagatccgagtgtggcacgacaacaaagggctcagccctgcctggttcctgcagcacgtcatcgtcagggacctgcagacggcacgcagcgccttcttcctggtcaatgactggctttcggtggagacggaggccaacgggggcctggtggagaaggaggtgctggccgcgagcgacgcagcccttttgcgcttccggcgcctgctggtggctgagctgcagcgtggcttctttgacaagcacatctggctctccatatgggaccggccgcctcgtagccgtttcactcgcatccagagggccacctgctgcgttctcctcatctgcctcttcctgggcgccaacgccgtgtggtacggggctgttggcgactctgcctacagcacggggcatgtgtccaggctgagcccgctgagcgtcgacacagtcgctgttggcctggtgtccagcgtggttgtctatcccgtctacctggccatcctttttctcttccggatgtcccggagcaaggtggctgggagcccgagccccacacctgccgggcagcaggtgctggacatcgacagctgcctggactcgtccgtgctggacagctccttcctcacgttctcaggcctccacgctgagcaggcctttgttggacagatgaagagtgacttgtttctggatgattctaagagtctggtgtgctggccctccggcgagggaacgctcagttggccggacctgctcagtgacccgtccattgtgggtagcaatctgcggcagctggcacggggccaggcgggccatgggctgggcccagaggaggacggcttctccctggccagcccctactcgcctgccaaatccttctcagcatcagatgaagacctgatccagcaggtccttgccgagggggtcagcagcccagcccctacccaagacacccacatggaaacggacctgctcagcagcctgtccagcactcctggggagaagacagagacgctggcgctgcagaggctgggggagctggggccacccagcccaggcctgaactgggaacagccccaggcagcgaggctgtccaggacaggactggtggagggtctgcggaagcgcctgctgccggcctggtgtgcctccctggcccacgggctcagcctgctcctggtggctgtggctgtggctgtctcagggtgggtgggtgcgagcttccccccgggcgtgagtgttgcgtggctcctgtccagcagcgccagcttcctggcctcattcctcggctgggagccactgaaggtcttgctggaagccctgtacttctcactggtggccaagcggctgcacccggatgaagatgacaccctggtagagagcccggctgtgacgcctgtgagcgcacgtgtgccccgcgtacggccaccccacggctttgcactcttcctggccaaggaagaagcccgcaaggtcaagaggctacatggcatgctgcggagcctcctggtgtacatgctttttctgctggtgaccctgctggccagctatggggatgcctcatgccatgggcacgcctaccgtctgcaaagcgccatcaagcaggagctgcacagccgggccttcctggccatcacgcggtctgaggagctctggccatggatggcccacgtgctgctgccctacgtccacgggaaccagtccagcccagagctggggcccccacggctgcggcaggtgcggctgcaggaagcactctacccagaccctcccggccccagggtccacacgtgctcggccgcaggaggcttcagcaccagcgattacgacgttggctgggagagtcctcacaatggctcggggacgtgggcctattcagcgccggatctgctgggggcatggtcctggggctcctgtgccgtgtatgacagcgggggctacgtgcaggagctgggcctgagcctggaggagagccgcgaccggctgcgcttcctgcagctgcacaactggctggacaacaggagccgcgctgtgttcctggagctcacgcgctacagcccggccgtggggctgcacgccgccgtcacgctgcgcctcgagttcccggcggccggccgcgccctggccgccctcagcgtccgcccctttgcgctgcgccgcctcagcgcgggcctctcgctgcctctgctcacctcggtgtgcctgctgctgttcgccgtgcacttcgccgtggccgaggcccgtacttggcacagggaagggcgctggcgcgtgctgcggctcggagcctgggcgcggtggctgctggtggcgctgacggcggccacggcactggtacgcctcgcccagctgggtgccgctgaccgccagtggacccgtttcgtgcgcggccgcccgcgccgcttcactagcttcgaccaggtggcgcagctgagctccgcagcccgtggcctggcggcctcgctgctcttcctgcttttggtcaaggctgcccagcagctacgcttcgtgcgccagtggtccgtctttggcaagacattatgccgagctctgccagagctcctgggggtcaccttgggcctggtggtgctcggggtagcctacgcccagctggccatcctgctcgtgtcttcctgtgtggactccctctggagcgtggcccaggccctgttggtgctgtgccctgggactgggctctctaccctgtgtcctgcctaa

SEQ ID NO: 15 - protein, 1230 aa, synthetic construct
MYIVMLTCAVCLVTYMVMAAILHKLDQLDASRGRAIPFCGQRGRFKYEILVKTGWGRGSGTTAHVGIMLYGVDSRSGHRHLDGDRAFHRNSLDIFRIATPHSLGSVWKIRVWHDNKGLSPAWFLQHVIVRDLQTARSAFFLVNDWLSVETEANGGLVEKEVLAASDAALLRFRRLLVAELQRGFFDKHIWLSIWDRPPRSRFTRIQRATCCVLLICLFLGANAVWYGAVGDSAYSTGHVSRLSPLSVDTVAVGLVSSVVVYPVYLAILFLFRMSRSKVAGSPSPTPAGQQVLDIDSCLDSSVLDSSFLTFSGLHAEQAFVGQMKSDLFLDDSKSLVCWPSGEGTLSWPDLLSDPSIVGSNLRQLARGQAGHGLGPEEDGFSLASPYSPAKSFSASDEDLIQQVLAEGVSSPAPTQDTHMETDLLSSLSSTPGEKTETLALQRLGELGPPSPGLNWEQPQAARLSRTGLVEGLRKRLLPAWCASLAHGLSLLLVAVAVAVSGWVGASFPPGVSVAWLLSSSASFLASFLGWEPLKVLLEALYFSLVAKRLHPDEDDTLVESPAVTPVSARVPRVRPPHGFALFLAKEEARKVKRLHGMLRSLLVYMLFLLVTLLASYGDASCHGHAYRLQSAIKQELHSRAFLAITRSEELWPWMAHVLLPYVHGNQSSPELGPPRLRQVRLQEALYPDPPGPRVHTCSAAGGFSTSDYDVGWESPHNGSGTWAYSAPDLLGAWSWGSCAVYDSGGYVQELGLSLEESRDRLRFLQLHNWLDNRSRAVFLELTRYSPAVGLHAAVTLRLEFPAAGRALAALSVRPFALRRLSAGLSLPLLTSVCLLLFAVHFAVAEARTWHREGRWRVLRLGAWARWLLVALTAATALVRLAQLGAADRQWTRFVRGRPRRFTSFDQVAQLSSAARGLAASLLFLLLVKAAQQLRFVRQWSVFGKTLCRALPELLGVTLGLVVLGVAYAQLAILLVSSCVDSLWSVAQALLVLCPGTGLSTLCPAESWHLSPLLCVGLWALRLWGALRLGAVILRWRYHALRGELYRPAWEPQDYEMVELFLRRLRLWMGLSKVKEFRHKVRFEGMEPLPSRSSRGSKVSPDVPPPSAGSDASHPSTSSSQLDGLSVSLGRLGTRCEPEPSRLQAVFEALLTQFDRLNQATEDVYQLEQQLHSLQGRRSSRAPAGSSRGPSPGLRPALPSRLARASRGVDLATGPSRTPLRAKNKVHPSST

SEQ ID NO: 16 - DNA, 3693 bp, synthetic construct
  source 1..3693: mol_type = other DNA
atgtacatcgtcatgctgacatgtgctgtgtgcctggtgacctacatggtcatggccgccatcctgcacaagctggaccagttggatgccagccggggccgcgccatccctttctgtgggcagcggggccgcttcaagtacgagatcctcgtcaagacaggctggggccggggctcaggtaccacggcccacgtgggcatcatgctgtatggggtggacagccggagcggccaccggcacctggacggcgacagagccttccaccgcaacagcctggacatcttccggatcgccaccccgcacagcctgggtagcgtgtggaagatccgagtgtggcacgacaacaaagggctcagccctgcctggttcctgcagcacgtcatcgtcagggacctgcagacggcacgcagcgccttcttcctggtcaatgactggctttcggtggagacggaggccaacgggggcctggtggagaaggaggtgctggccgcgagcgacgcagcccttttgcgcttccggcgcctgctggtggctgagctgcagcgtggcttctttgacaagcacatctggctctccatatgggaccggccgcctcgtagccgtttcactcgcatccagagggccacctgctgcgttctcctcatctgcctcttcctgggcgccaacgccgtgtggtacggggctgttggcgactctgcctacagcacggggcatgtgtccaggctgagcccgctgagcgtcgacacagtcgctgttggcctggtgtccagcgtggttgtctatcccgtctacctggccatcctttttctcttccggatgtcccggagcaaggtggctgggagcccgagccccacacctgccgggcagcaggtgctggacatcgacagctgcctggactcgtccgtgctggacagctccttcctcacgttctcaggcctccacgctgagcaggcctttgttggacagatgaagagtgacttgtttctggatgattctaagagtctggtgtgctggccctccggcgagggaacgctcagttggccggacctgctcagtgacccgtccattgtgggtagcaatctgcggcagctggcacggggccaggcgggccatgggctgggcccagaggaggacggcttctccctggccagcccctactcgcctgccaaatccttctcagcatcagatgaagacctgatccagcaggtccttgccgagggggtcagcagcccagcccctacccaagacacccacatggaaacggacctgctcagcagcctgtccagcactcctggggagaagacagagacgctggcgctgcagaggctgggggagctggggccacccagcccaggcctgaactgggaacagccccaggcagcgaggctgtccaggacaggactggtggagggtctgcggaagcgcctgctgccggcctggtgtgcctccctggcccacgggctcagcctgctcctggtggctgtggctgtggctgtctcagggtgggtgggtgcgagcttccccccgggcgtgagtgttgcgtggctcctgtccagcagcgccagcttcctggcctcattcctcggctgggagccactgaaggtcttgctggaagccctgtacttctcactggtggccaagcggctgcacccggatgaagatgacaccctggtagagagcccggctgtgacgcctgtgagcgcacgtgtgccccgcgtacggccaccccacggctttgcactcttcctggccaaggaagaagcccgcaaggtcaagaggctacatggcatgctgcggagcctcctggtgtacatgctttttctgctggtgaccctgctggccagctatggggatgcctcatgccatgggcacgcctaccgtctgcaaagcgccatcaagcaggagctgcacagccgggccttcctggccatcacgcggtctgaggagctctggccatggatggcccacgtgctgctgccctacgtccacgggaaccagtccagcccagagctggggcccccacggctgcggcaggtgcggctgcaggaagcactctacccagaccctcccggccccagggtccacacgtgctcggccgcaggaggcttcagcaccagcgattacgacgttggctgggagagtcctcacaatggctcggggacgtgggcctattcagcgccggatctgctgggggcatggtcctggggctcctgtgccgtgtatgacagcgggggctacgtgcaggagctgggcctgagcctggaggagagccgcgaccggctgcgcttcctgcagctgcacaactggctggacaacaggagccgcgctgtgttcctggagctcacgcgctacagcccggccgtggggctgcacgccgccgtcacgctgcgcctcgagttcccggcggccggccgcgccctggccgccctcagcgtccgcccctttgcgctgcgccgcctcagcgcgggcctctcgctgcctctgctcacctcggtgtgcctgctgctgttcgccgtgcacttcgccgtggccgaggcccgtacttggcacagggaagggcgctggcgcgtgctgcggctcggagcctgggcgcggtggctgctggtggcgctgacggcggccacggcactggtacgcctcgcccagctgggtgccgctgaccgccagtggacccgtttcgtgcgcggccgcccgcgccgcttcactagcttcgaccaggtggcgcagctgagctccgcagcccgtggcctggcggcctcgctgctcttcctgcttttggtcaaggctgcccagcagctacgcttcgtgcgccagtggtccgtctttggcaagacattatgccgagctctgccagagctcctgggggtcaccttgggcctggtggtgctcggggtagcctacgcccagctggccatcctgctcgtgtcttcctgtgtggactccctctggagcgtggcccaggccctgttggtgctgtgccctgggactgggctctctaccctgtgtcctgccgagtcctggcacctgtcacccctgctgtgtgtggggctctgggcactgcggctgtggggcgccctacggctgggggctgttattctccgctggcgctaccacgccttgcgtggagagctgtaccggccggcctgggagccccaggactacgagatggtggagttgttcctgcgcaggctgcgcctctggatgggcctcagcaaggtcaaggagttccgccacaaagtccgctttgaagggatggagccgctgccctctcgctcctccaggggctccaaggtatccccggatgtgcccccacccagcgctggctccgatgcctcgcacccctccacctcctccagccagctggatgggctgagcgtgagcctgggccggctggggacaaggtgtgagcctgagccctcccgcctccaagccgtgttcgaggccctgctcacccagtttgaccgactcaaccaggccacagaggacgtctaccagctggagcagcagctgcacagcctgcaaggccgcaggagcagccgggcgcccgccggatcttcccgtggcccatccccgggcctgcggccagcactgcccagccgccttgcccgggccagtcggggtgtggacctggccactggccccagcaggacaccccttcgggccaagaacaaggtccaccccagcagcacttaa

SEQ ID NO: 17 - protein, 703 aa, synthetic construct
MGWEPLKVLLEALYFSLVAKRLHPDEDDTLVESPAVTPVSARVPRVRPPHGFALFLAKEEARKVKRLHGMLRSLLVYMLFLLVTLLASYGDASCHGHAYRLQSAIKQELHSRAFLAITRSEELWPWMAHVLLPYVHGNQSSPELGPPRLRQVRLQEALYPDPPGPRVHTCSAAGGFSTSDYDVGWESPHNGSGTWAYSAPDLLGAWSWGSCAVYDSGGYVQELGLSLEESRDRLRFLQLHNWLDNRSRAVFLELTRYSPAVGLHAAVTLRLEFPAAGRALAALSVRPFALRRLSAGLSLPLLTSVCLLLFAVHFAVAEARTWHREGRWRVLRLGAWARWLLVALTAATALVRLAQLGAADRQWTRFVRGRPRRFTSFDQVAQLSSAARGLAASLLFLLLVKAAQQLRFVRQWSVFGKTLCRALPELLGVTLGLVVLGVAYAQLAILLVSSCVDSLWSVAQALLVLCPGTGLSTLCPAESWHLSPLLCVGLWALRLWGALRLGAVILRWRYHALRGELYRPAWEPQDYEMVELFLRRLRLWMGLSKVKEFRHKVRFEGMEPLPSRSSRGSKVSPDVPPPSAGSDASHPSTSSSQLDGLSVSLGRLGTRCEPEPSRLQAVFEALLTQFDRLNQATEDVYQLEQQLHSLQGRRSSRAPAGSSRGPSPGLRPALPSRLARASRGVDLATGPSRTPLRAKNKVHPSST

SEQ ID NO: 18 - DNA, 2112 bp, synthetic construct
  source 1..2112: mol_type = other DNA
atgggctgggagccactgaaggtcttgctggaagccctgtacttctcactggtggccaagcggctgcacccggatgaagatgacaccctggtagagagcccggctgtgacgcctgtgagcgcacgtgtgccccgcgtacggccaccccacggctttgcactcttcctggccaaggaagaagcccgcaaggtcaagaggctacatggcatgctgcggagcctcctggtgtacatgctttttctgctggtgaccctgctggccagctatggggatgcctcatgccatgggcacgcctaccgtctgcaaagcgccatcaagcaggagctgcacagccgggccttcctggccatcacgcggtctgaggagctctggccatggatggcccacgtgctgctgccctacgtccacgggaaccagtccagcccagagctggggcccccacggctgcggcaggtgcggctgcaggaagcactctacccagaccctcccggccccagggtccacacgtgctcggccgcaggaggcttcagcaccagcgattacgacgttggctgggagagtcctcacaatggctcggggacgtgggcctattcagcgccggatctgctgggggcatggtcctggggctcctgtgccgtgtatgacagcgggggctacgtgcaggagctgggcctgagcctggaggagagccgcgaccggctgcgcttcctgcagctgcacaactggctggacaacaggagccgcgctgtgttcctggagctcacgcgctacagcccggccgtggggctgcacgccgccgtcacgctgcgcctcgagttcccggcggccggccgcgccctggccgccctcagcgtccgcccctttgcgctgcgccgcctcagcgcgggcctctcgctgcctctgctcacctcggtgtgcctgctgctgttcgccgtgcacttcgccgtggccgaggcccgtacttggcacagggaagggcgctggcgcgtgctgcggctcggagcctgggcgcggtggctgctggtggcgctgacggcggccacggcactggtacgcctcgcccagctgggtgccgctgaccgccagtggacccgtttcgtgcgcggccgcccgcgccgcttcactagcttcgaccaggtggcgcagctgagctccgcagcccgtggcctggcggcctcgctgctcttcctgcttttggtcaaggctgcccagcagctacgcttcgtgcgccagtggtccgtctttggcaagacattatgccgagctctgccagagctcctgggggtcaccttgggcctggtggtgctcggggtagcctacgcccagctggccatcctgctcgtgtcttcctgtgtggactccctctggagcgtggcccaggccctgttggtgctgtgccctgggactgggctctctaccctgtgtcctgccgagtcctggcacctgtcacccctgctgtgtgtggggctctgggcactgcggctgtggggcgccctacggctgggggctgttattctccgctggcgctaccacgccttgcgtggagagctgtaccggccggcctgggagccccaggactacgagatggtggagttgttcctgcgcaggctgcgcctctggatgggcctcagcaaggtcaaggagttccgccacaaagtccgctttgaagggatggagccgctgccctctcgctcctccaggggctccaaggtatccccggatgtgcccccacccagcgctggctccgatgcctcgcacccctccacctcctccagccagctggatgggctgagcgtgagcctgggccggctggggacaaggtgtgagcctgagccctcccgcctccaagccgtgttcgaggccctgctcacccagtttgaccgactcaaccaggccacagaggacgtctaccagctggagcagcagctgcacagcctgcaaggccgcaggagcagccgggcgcccgccggatcttcccgtggcccatccccgggcctgcggccagcactgcccagccgccttgcccgggccagtcggggtgtggacctggccactggccccagcaggacaccccttcgggccaagaacaaggtccaccccagcagcacttaa

SEQ ID NO: 19 - protein, 723 aa, synthetic construct
METDTLLLWVLLLWVPGSTGDGWEPLKVLLEALYFSLVAKRLHPDEDDTLVESPAVTPVSARVPRVRPPHGFALFLAKEEARKVKRLHGMLRSLLVYMLFLLVTLLASYGDASCHGHAYRLQSAIKQELHSRAFLAITRSEELWPWMAHVLLPYVHGNQSSPELGPPRLRQVRLQEALYPDPPGPRVHTCSAAGGFSTSDYDVGWESPHNGSGTWAYSAPDLLGAWSWGSCAVYDSGGYVQELGLSLEESRDRLRFLQLHNWLDNRSRAVFLELTRYSPAVGLHAAVTLRLEFPAAGRALAALSVRPFALRRLSAGLSLPLLTSVCLLLFAVHFAVAEARTWHREGRWRVLRLGAWARWLLVALTAATALVRLAQLGAADRQWTRFVRGRPRRFTSFDQVAQLSSAARGLAASLLFLLLVKAAQQLRFVRQWSVFGKTLCRALPELLGVTLGLVVLGVAYAQLAILLVSSCVDSLWSVAQALLVLCPGTGLSTLCPAESWHLSPLLCVGLWALRLWGALRLGAVILRWRYHALRGELYRPAWEPQDYEMVELFLRRLRLWMGLSKVKEFRHKVRFEGMEPLPSRSSRGSKVSPDVPPPSAGSDASHPSTSSSQLDGLSVSLGRLGTRCEPEPSRLQAVFEALLTQFDRLNQATEDVYQLEQQLHSLQGRRSSRAPAGSSRGPSPGLRPALPSRLARASRGVDLATGPSRTPLRAKNKVHPSST

SEQ ID NO: 20 - DNA, 2172 bp, synthetic construct
  source 1..2172: mol_type = other DNA
atggagacagacacactcctgctatgggtactgctgctctgggttccaggttccactggtgacggctgggagccactgaaggtcttgctggaagccctgtacttctcactggtggccaagcggctgcacccggatgaagatgacaccctggtagagagcccggctgtgacgcctgtgagcgcacgtgtgccccgcgtacggccaccccacggctttgcactcttcctggccaaggaagaagcccgcaaggtcaagaggctacatggcatgctgcggagcctcctggtgtacatgctttttctgctggtgaccctgctggccagctatggggatgcctcatgccatgggcacgcctaccgtctgcaaagcgccatcaagcaggagctgcacagccgggccttcctggccatcacgcggtctgaggagctctggccatggatggcccacgtgctgctgccctacgtccacgggaaccagtccagcccagagctggggcccccacggctgcggcaggtgcggctgcaggaagcactctacccagaccctcccggccccagggtccacacgtgctcggccgcaggaggcttcagcaccagcgattacgacgttggctgggagagtcctcacaatggctcggggacgtgggcctattcagcgccggatctgctgggggcatggtcctggggctcctgtgccgtgtatgacagcgggggctacgtgcaggagctgggcctgagcctggaggagagccgcgaccggctgcgcttcctgcagctgcacaactggctggacaacaggagccgcgctgtgttcctggagctcacgcgctacagcccggccgtggggctgcacgccgccgtcacgctgcgcctcgagttcccggcggccggccgcgccctggccgccctcagcgtccgcccctttgcgctgcgccgcctcagcgcgggcctctcgctgcctctgctcacctcggtgtgcctgctgctgttcgccgtgcacttcgccgtggccgaggcccgtacttggcacagggaagggcgctggcgcgtgctgcggctcggagcctgggcgcggtggctgctggtggcgctgacggcggccacggcactggtacgcctcgcccagctgggtgccgctgaccgccagtggacccgtttcgtgcgcggccgcccgcgccgcttcactagcttcgaccaggtggcgcagctgagctccgcagcccgtggcctggcggcctcgctgctcttcctgcttttggtcaaggctgcccagcagctacgcttcgtgcgccagtggtccgtctttggcaagacattatgccgagctctgccagagctcctgggggtcaccttgggcctggtggtgctcggggtagcctacgcccagctggccatcctgctcgtgtcttcctgtgtggactccctctggagcgtggcccaggccctgttggtgctgtgccctgggactgggctctctaccctgtgtcctgccgagtcctggcacctgtcacccctgctgtgtgtggggctctgggcactgcggctgtggggcgccctacggctgggggctgttattctccgctggcgctaccacgccttgcgtggagagctgtaccggccggcctgggagccccaggactacgagatggtggagttgttcctgcgcaggctgcgcctctggatgggcctcagcaaggtcaaggagttccgccacaaagtccgctttgaagggatggagccgctgccctctcgctcctccaggggctccaaggtatccccggatgtgcccccacccagcgctggctccgatgcctcgcacccctccacctcctccagccagctggatgggctgagcgtgagcctgggccggctggggacaaggtgtgagcctgagccctcccgcctccaagccgtgttcgaggccctgctcacccagtttgaccgactcaaccaggccacagaggacgtctaccagctggagcagcagctgcacagcctgcaaggccgcaggagcagccgggcgcccgccggatcttcccgtggcccatccccgggcctgcggccagcactgcccagccgccttgcccgggccagtcggggtgtggacctggccactggccccagcaggacaccccttcgggccaagaacaaggtccaccccagcagcacttaa

SEQ ID NO: 21 - protein, 493 aa, synthetic construct
MWQLLLPTALLLLVSAGMRTEDLPKAVVFLEPQWYSVLEKDSVTLKCQGAYSPEDNSTQWFHNESLISSQASSYFIDAATVNDSGEYRCQTNLSTLSDPVQLEVHIGWLLLQAPRWVFKEEDPIHLRCHSWKNTALHKVTYLQNGKDRKYFHHNSDFHIPKATLKDSGSYFCRGLVGSKNVSSETVNITITQGLAVSTISSFSPPGADPPRASALPAPPTGSALPDPQTASALPDPPAASALPAALAVISFLLGLGLGVACVLARTRESWHLSPLLCVGLWALRLWGALRLGAVILRWRYHALRGELYRPAWEPQDYEMVELFLRRLRLWMGLSKVKEFRHKVRFEGMEPLPSRSSRGSKVSPDVPPPSAGSDASHPSTSSSQLDGLSVSLGRLGTRCEPEPSRLQAVFEALLTQFDRLNQATEDVYQLEQQLHSLQGRRSSRAPAGSSRGPSPGLRPALPSRLARASRGVDLATGPSRTPLRAKNKVHPSST

SEQ ID NO: 22 - DNA, 1482 bp, synthetic construct
  source 1..1482: mol_type = other DNA
atgtggcagctgctcctcccaactgctctgctacttctagtttcagctggcatgcggactgaagatctcccaaaggctgtggtgttcctggagcctcaatggtacagcgtgcttgagaaggacagtgtgactctgaagtgccagggagcctactcccctgaggacaattccacacagtggtttcacaatgagagcctcatctcaagccaggcctcgagctacttcattgacgctgccacagtcaacgacagtggagagtacaggtgccagacaaacctctccaccctcagtgacccggtgcagctagaagtccatatcggctggctgttgctccaggcccctcggtgggtgttcaaggaggaagaccctattcacctgaggtgtcacagctggaagaacactgctctgcataaggtcacatatttacagaatggcaaagacaggaagtattttcatcataattctgacttccacattccaaaagccacactcaaagatagcggctcctacttctgcagggggcttgttgggagtaaaaatgtgtcttcagagactgtgaacatcaccatcactcaaggtttggcagtgtcaaccatctcatcattctctccacctggcgcggatccaccaagggcctctgccctccctgccccaccgacaggctccgccctccctgacccgcagacagcctctgccctccctgacccgccagcagcctctgccctccctgcggccctggcggtgatctccttcctcctcgggctgggcctgggggtggcgtgtgtgctggcgaggacgcgtgagtcctggcacttgtcacccctgctgtgtgtggggctctgggcactgcggctgtggggcgccctacggctgggggctgttattctccgctggcgctaccacgccttgcgtggagagctgtaccggccggcctgggagccccaggactacgagatggtggagttgttcctgcgcaggctgcgcctctggatgggcctcagcaaggtcaaggagttccgccacaaagtccgctttgaagggatggagccgctgccctctcgctcctccaggggctccaaggtatccccggatgtgcccccacccagcgctggctccgatgcctcgcacccctccacctcctccagccagctggatgggctgagcgtgagcctgggccggctggggacaaggtgtgagcctgagccctcccgcctccaagccgtgttcgaggccctgctcacccagtttgaccgactcaaccaggccacagaggacgtctaccagctggagcagcagctgcacagcctgcaaggccgcaggagcagccgggcgcccgccggatcttcccgtggcccatccccgggcctgcggccagcactgcccagccgccttgcccgggccagtcggggtgtggacctggccactggccccagcaggacaccccttcgggccaagaacaaggtccaccccagcagcacttag

SEQ ID NO: 23 - DNA, 3771 bp, synthetic construct
  source 1..3771: mol_type = other DNA
atgagtgctgctggggtggaccttgttcttggcccgaaggggtgtcctgctggggccagtggccaggtccacaccccgactggcccgggcaaggcggctgggcagtgctggccgcaggcccggggatgggccacgggaagatccggcgggcgcccggctgctcctgcggccttgcaggctgtgcagctgctgctccagctggtagacgtcctctgtggcctggttgagtcggtcaaactgggtgagcagggcctcgaacacggcttggaggcgggagggctcaggctcacaccttgtccccagccggcccaggctcacgctcagcccatccagctggctggaggaggtggaggggtgcgaggcatcggagccagcgctgggtgggggcacatccggggataccttggagcccctggaggagcgagagggcagcggctccatcccttcaaagcggactttgtggcggaactccttgaccttgctgaggcccatccagaggcgcagcctgcgcaggaacaactccaccatctcgtagtcctggggctcccaggccggccggtacagctctccacgcaaggcgtggtagcgccagcggagaataacagcccccagccgtagggcgccccacagccgcagtgcccagagccccacacacagcaggggtgacaggtgccaggactcggcaggacacagggtagagagcccagtcccagggcacagcaccaacagggcctgggccacgctccagagggagtccacacaggaagacacgagcaggatggccagctgggcgtaggctaccccgagcaccaccaggcccaaggtgacccccaggagctctggcagagctcggcataatgtcttgccaaagacggaccactggcgcacgaagcgtagctgctgggcagccttgaccaaaagcaggaagagcagcgaggccgccaggccacgggctgcggagctcagctgcgccacctggtcgaagctagtgaagcggcgcgggcggccgcgcacgaaacgggtccactggcggtcagcggcacccagctgggcgaggcgtaccagtgccgtggccgccgtcagcgccaccagcagccaccgcgcccaggctccgagccgcagcacgcgccagcgcccttccctgtgccaagtacgggcctcggccacggcgaagtgcacggcgaacagcagcaggcacaccgaggtgagcagaggcagcgagaggcccgcgctgaggcggcgcagcgcaaaggggcggacgctgagggcggccagggcgcggccggccgccgggaactcgaggcgcagcgtgacggcggcgtgcagccccacggccgggctgtagcgcgtgagctccaggaacacagcgcggctcctgttgtccagccagttgtgcagctgcaggaagcgcagccggtcgcggctctcctccaggctcaggcccagctcctgcacgtagcccccgctgtcatacacggcacaggagccccaggaccatgcccccagcagatccggcgctgaataggcccacgtccccgagccattgtgaggactctcccagccaacgtcgtaatcgctggtgctgaagcctcctgcggccgagcacgtgtggaccctggggccgggagggtctgggtagagtgcttcctgcagccgcacctgccgcagccgtgggggccccagctctgggctggactggttcccgtggacgtagggcagcagcacgtgggccatccatggccagagctcctcagaccgcgtgatggccaggaaggcccggctgtgcagctcctgcttgatggcgctttgcagacggtaggcgtgcccatggcatgaggcatccccatagctggccagcagggtcaccagcagaaaaagcatgtacaccaggaggctccgcagcatgccatgtagcctcttgaccttgcgggcttcttccttggccaggaagagtgcaaagccgtggggtggccgtacgcggggcacacgtgcgctcacaggcgtcacagccgggctctctaccagggtgtcatcttcatccgggtgcagccgcttggccaccagtgagaagtacagggcttccagcaagaccttcagtggctcccagccgaggaatgaggccaggaagctggcgctgctggacaggagccacgcaacactcacgcccggggggaagctcgcacccacccaccctgagacagccacagccacagccaccaggagcaggctgagcccgtgggccagggaggcacaccaggccggcagcaggcgcttccgcagaccctccaccagtcctgtcctggacagcctcgctgcctggggctgttcccagttcaggcctgggctgggtggccccagctcccccagcctctgcagcgccagcgtctctgtcttctccccaggagtgctggacaggctgctgagcaggtccgtttccatgtgggtgtcttgggtaggggctgggctgctgaccccctcggcaaggacctgctggatcaggtcttcatctgatgctgagaaggatttggcaggcgagtaggggctggccagggagaagccgtcctcctctgggcccagcccatggcccgcctggccccgtgccagctgccgcagattgctacccacaatggacgggtcactgagcaggtccggccaactgagcgttccctcgccggagggccagcacaccagactcttagaatcatccagaaacaagtcactcttcatctgtccaacaaaggcctgctcagcgtggaggcctgagaacgtgaggaaggagctgtccagcacggacgagtccaggcagctgtcgatgtccagcacctgctgcccggcaggtgtggggctcgggctcccagccaccttgctccgggacatccggaagagaaaaaggatggccaggtagacgggatagacaaccacgctggacaccaggccaacagcgactgtgtcgacgctcagcgggctcagcctggacacatgccccgtgctgtaggcagagtcgccaacagccccgtaccacacggcgttggcgcccaggaagaggcagatgaggagaacgcagcaggtggccctctggatgcgagtgaaacggctacgaggcggccggtcccatatggagagccagatgtgcttgtcaaagaagccacgctgcagctcagccaccagcaggcgccggaagcgcaaaagggctgcgtcgctcgcggccagcacctccttctccaccaggcccccgttggcctccgtctccaccgaaagccagtcattgaccaggaagaaggcgctgcgtgccgtctgcaggtccctgacgatgacgtgctgcaggaaccaggcagggctgagccctttgttgtcgtgccacactcggatcttccacacgctacccaggctgtgcggggtggcgatccggaagatgtccaggctgttgcggtggaaggctctgtcgccgtccaggtgccggtggccgctccggctgtccaccccatacagcatgatgcccacgtgggccgtggtacctgagccccggccccagcctgtcttgacgaggatctcgtacttgaagcggccccgctgcccacagaaagggatggcgcggccccggctggcatccaactggtccagcttgtgcaggatggcggccatgaccatgtaggtcaccaggcacacagcacatgtcagcatgacgatgtagtttacatccgctgtcggctcaggaaacacaaagcggacatggcttgggggcacgaagaggctggcgccgaaggcggttaa

SEQ ID NO: 24 - protein, 390 aa, synthetic construct
MLGIWTLLPLVLTSVARLSSKSVNAQVTDINSKGLELRKTVTTVETQNLEGLHHDGQFCHKPCPPGERKARDCTVNGDEPDCVPCQEGKEYTDKAHFSSKCRRCRLCDEGHGLEVEINCTRTQNTKCRCKPNFFCNSTVCEHCDPCTKCEHGIIKECTLTSNTKCKEEGSRSNLGWLCLLLLPIPLIVWVVILRWRYHALRGELYRPAWEPQDYEMVELFLRRLRLWMGLSKVKEFRHKVRFEGMEPLPSRSSRGSKVSPDVPPPSAGSDASHPSTSSSQLDGLSVSLGRLGTRCEPEPSRLQAVFEALLTQFDRLNQATEDVYQLEQQLHSLQGRRSSRAPAGSSRGPSPGLRPALPSRLARASRGVDLATGPSRTPLRAKNKVHPSST

SEQ ID NO: 25 - DNA, 1173 bp, synthetic construct
  source 1..1173: mol_type = other DNA
atgctgggcatctggaccctcctacctctggttcttacgtctgttgctagattatcgtccaaaagtgttaatgcccaagtgactgacatcaactccaagggattggaattgaggaagactgttactacagttgagactcagaacttggaaggcctgcatcatgatggccaattctgccataagccctgtcctccaggtgaaaggaaagctagggactgcacagtcaatggggatgaaccagactgcgtgccctgccaagaagggaaggagtacacagacaaagcccatttttcttccaaatgcagaagatgtagattgtgtgatgaaggacatggcttagaagtggaaataaactgcacccggacccagaataccaagtgcagatgtaaaccaaactttttttgtaactctactgtatgtgaacactgtgacccttgcaccaaatgtgaacatggaatcatcaaggaatgcacactcaccagcaacaccaagtgcaaagaggaaggatccagatctaacttggggtggctttgtcttcttcttttgccaattccactaattgtttgggtggttattctccgctggcgctaccacgccttgcgtggagagctgtaccggccggcctgggagccccaggactacgagatggtggagttgttcctgcgcaggctgcgcctctggatgggcctcagcaaggtcaaggagttccgccacaaagtccgctttgaagggatggagccgctgccctctcgctcctccaggggctccaaggtatccccggatgtgcccccacccagcgctggctccgatgcctcgcacccctccacctcctccagccagctggatgggctgagcgtgagcctgggccggctggggacaaggtgtgagcctgagccctcccgcctccaagccgtgttcgaggccctgctcacccagtttgaccgactcaaccaggccacagaggacgtctaccagctggagcagcagctgcacagcctgcaaggccgcaggagcagccgggcgcccgccggatcttcccgtggcccatccccgggcctgcggccagcactgcccagccgccttgcccgggccagtcggggtgtggacctggccactggccccagcaggacaccccttcgggccaagaacaaggtccaccccagcagcacttag

SEQ ID NO: 26 - protein, 180 aa, synthetic construct
MVILRWRYHALRGELYRPAWEPQDYEMVELFFEGMEPLPSRSSRGSKVSPDVPPPSAGSDASHPSTSSSQLDGLSVSLGRLGTRCEPEPSRLQAVFEALLTQFDRLNQATEDVYQLEQQLHSLQGRRSSRAPAGSSRGPSPGLRPALPSRLARASRGVDLATGPSRTPLRAKNKVHPSST

SEQ ID NO: 27 - DNA, 543 bp, synthetic construct
  source 1..543: mol_type = other DNA
atggttattctccgctggcgctaccacgccttgcgtggagagctgtaccggccggcctgggagccccaggactacgagatggtggagttgttctttgaagggatggagccgctgccctctcgctcctccaggggctccaaggtatccccggatgtgcccccacccagcgctggctccgatgcctcgcacccctccacctcctccagccagctggatgggctgagcgtgagcctgggccggctggggacaaggtgtgagcctgagccctcccgcctccaagccgtgttcgaggccctgctcacccagtttgaccgactcaaccaggccacagaggacgtctaccagctggagcagcagctgcacagcctgcaaggccgcaggagcagccgggcgcccgccggatcttcccgtggcccatccccgggcctgcggccagcactgcccagccgccttgcccgggccagtcggggtgtggacctggccactggccccagcaggacaccccttcgggccaagaacaaggtccaccccagcagcacttag

SEQ ID NO: 28 - protein, 101 aa, synthetic construct
MVILRWRYHALRGELYRPAWEPQDYEMVELFLRRLRLWMGLSKVKEFRHKVRFEGMEPLPSRSSRGSKVSPDVPPPSAGSDASHPSTSSSQLDGLSVSLGR

SEQ ID NO: 29 - DNA, 306 bp, synthetic construct
  source 1..306: mol_type = other DNA
atggttattctccgctggcgctaccacgccttgcgtggagagctgtaccggccggcctgggagccccaggactacgagatggtggagttgttcctgcgcaggctgcgcctctggatgggcctcagcaaggtcaaggagttccgccacaaagtccgctttgaagggatggagccgctgccctctcgctcctccaggggctccaaggtatccccggatgtgcccccacccagcgctggctccgatgcctcgcacccctccacctcctccagccagctggatgggctgagcgtgagcctgggccggtag

SEQ ID NO: 30 - protein, 101 aa, synthetic construct
MRFEGMEPLPSRSSRGSKVSPDVPPPSAGSDASHPSTSSSQLDGLSVSLGRLGTRCEPEPSRLQAVFEALLTQFDRLNQATEDVYQLEQQLHSLQGRRSSR

SEQ ID NO: 31 - DNA, 306 bp, synthetic construct
  source 1..306: mol_type = other DNA
atgcgctttgaagggatggagccgctgccctctcgctcctccaggggctccaaggtatccccggatgtgcccccacccagcgctggctccgatgcctcgcacccctccacctcctccagccagctggatgggctgagcgtgagcctgggccggctggggacaaggtgtgagcctgagccctcccgcctccaagccgtgttcgaggccctgctcacccagtttgaccgactcaaccaggccacagaggacgtctaccagctggagcagcagctgcacagcctgcaaggccgcaggagcagccggtag

SEQ ID NO: 32 - protein, 112 aa, synthetic construct
MQLDGLSVSLGRLGTRCEPEPSRLQAVFEALLTQFDRLNQATEDVYQLEQQLHSLQGRRSSRAPAGSSRGPSPGLRPALPSRLARASRGVDLATGPSRTPLRAKNKVHPSST

SEQ ID NO: 33 - DNA, 339 bp, synthetic construct
  source 1..339: mol_type = other DNA
atgcagctggatgggctgagcgtgagcctgggccggctggggacaaggtgtgagcctgagccctcccgcctccaagccgtgttcgaggccctgctcacccagtttgaccgactcaaccaggccacagaggacgtctaccagctggagcagcagctgcacagcctgcaaggccgcaggagcagccgggcgcccgccggatcttcccgtggcccatccccgggcctgcggccagcactgcccagccgccttgcccgggccagtcggggtgtggacctggccactggccccagcaggacaccccttcgggccaagaacaaggtccaccccagcagcacttag

SEQ ID NO: 34 - protein, 101 aa, synthetic construct
MLGTRCEPEPSRLQAVFEALLTQFDRLNQATEDVYQLEQQLHSLQGRRSSRAPAGSSRGPSPGLRPALPSRLARASRGVDLATGPSRTPLRAKNKVHPSST

SEQ ID NO: 35 - DNA, 306 bp, synthetic construct
  source 1..306: mol_type = other DNA
atgctggggacaaggtgtgagcctgagccctcccgcctccaagccgtgttcgaggccctgctcacccagtttgaccgactcaaccaggccacagaggacgtctaccagctggagcagcagctgcacagcctgcaaggccgcaggagcagccgggcgcccgccggatcttcccgtggcccatccccgggcctgcggccagcactgcccagccgccttgcccgggccagtcggggtgtggacctggccactggccccagcaggacaccccttcgggccaagaacaaggtccaccccagcagcacttag

SEQ ID NO: 36 - protein, 446 aa, synthetic construct
MWQLLLPTALLLLVSAGMRTEDLPKAVVFLEPQWYSVLEKDSVTLKCQGAYSPEDNSTQWFHNESLISSQASSYFIDAATVNDSGEYRCQTNLSTLSDPVQLEVHIGWLLLQAPRWVFKEEDPIHLRCHSWKNTALHKVTYLQNGKDRKYFHHNSDFHIPKATLKDSGSYFCRGLVGSKNVSSETVNITITQGLAVSTISSFSPPGADPPRASALPAPPTGSALPDPQTASALPDPPAASALPAALAVISFLLGLGLGVACVLARTRVILRWRYHALRGELYRPAWEPQDYEMVELFFEGMEPLPSRSSRGSKVSPDVPPPSAGSDASHPSTSSSQLDGLSVSLGRLGTRCEPEPSRLQAVFEALLTQFDRLNQATEDVYQLEQQLHSLQGRRSSRAPAGSSRGPSPGLRPALPSRLARASRGVDLATGPSRTPLRAKNKVHPSST

SEQ ID NO: 37 - DNA, 1341 bp, synthetic construct
  source 1..1341: mol_type = other DNA
atgtggcagctgctcctcccaactgctctgctacttctagtttcagctggcatgcggactgaagatctcccaaaggctgtggtgttcctggagcctcaatggtacagcgtgcttgagaaggacagtgtgactctgaagtgccagggagcctactcccctgaggacaattccacacagtggtttcacaatgagagcctcatctcaagccaggcctcgagctacttcattgacgctgccacagtcaacgacagtggagagtacaggtgccagacaaacctctccaccctcagtgacccggtgcagctagaagtccatatcggctggctgttgctccaggcccctcggtgggtgttcaaggaggaagaccctattcacctgaggtgtcacagctggaagaacactgctctgcataaggtcacatatttacagaatggcaaagacaggaagtattttcatcataattctgacttccacattccaaaagccacactcaaagatagcggctcctacttctgcagggggcttgttgggagtaaaaatgtgtcttcagagactgtgaacatcaccatcactcaaggtttggcagtgtcaaccatctcatcattctctccacctggcgcggatccaccaagggcctctgccctccctgccccaccgacaggctccgccctccctgacccgcagacagcctctgccctccctgacccgccagcagcctctgccctccctgcggccctggcggtgatctccttcctcctcgggctgggcctgggggtggcgtgtgtgctggcgaggacgcgtgttattctccgctggcgctaccacgccttgcgtggagagctgtaccggccggcctgggagccccaggactacgagatggtggagttgttctttgaagggatggagccgctgccctctcgctcctccaggggctccaaggtatccccggatgtgcccccacccagcgctggctccgatgcctcgcacccctccacctcctccagccagctggatgggctgagcgtgagcctgggccggctggggacaaggtgtgagcctgagccctcccgcctccaagccgtgttcgaggccctgctcacccagtttgaccgactcaaccaggccacagaggacgtctaccagctggagcagcagctgcacagcctgcaaggccgcaggagcagccgggcgcccgccggatcttcccgtggcccatccccgggcctgcggccagcactgcccagccgccttgcccgggccagtcggggtgtggacctggccactggccccagcaggacaccccttcgggccaagaacaaggtccaccccagcagcacttaa

SEQ ID NO: 38 - protein, 367 aa, synthetic construct
MWQLLLPTALLLLVSAGMRTEDLPKAVVFLEPQWYSVLEKDSVTLKCQGAYSPEDNSTQWFHNESLISSQASSYFIDAATVNDSGEYRCQTNLSTLSDPVQLEVHIGWLLLQAPRWVFKEEDPIHLRCHSWKNTALHKVTYLQNGKDRKYFHHNSDFHIPKATLKDSGSYFCRGLVGSKNVSSETVNITITQGLAVSTISSFSPPGADPPRASALPAPPTGSALPDPQTASALPDPPAASALPAALAVISFLLGLGLGVACVLARTRVILRWRYHALRGELYRPAWEPQDYEMVELFLRRLRLWMGLSKVKEFRHKVRFEGMEPLPSRSSRGSKVSPDVPPPSAGSDASHPSTSSSQLDGLSVSLGR

SEQ ID NO: 39 - DNA, 1104 bp, synthetic construct
  source 1..1104: mol_type = other DNA
atgtggcagctgctcctcccaactgctctgctacttctagtttcagctggcatgcggactgaagatctcccaaaggctgtggtgttcctggagcctcaatggtacagcgtgcttgagaaggacagtgtgactctgaagtgccagggagcctactcccctgaggacaattccacacagtggtttcacaatgagagcctcatctcaagccaggcctcgagctacttcattgacgctgccacagtcaacgacagtggagagtacaggtgccagacaaacctctccaccctcagtgacccggtgcagctagaagtccatatcggctggctgttgctccaggcccctcggtgggtgttcaaggaggaagaccctattcacctgaggtgtcacagctggaagaacactgctctgcataaggtcacatatttacagaatggcaaagacaggaagtattttcatcataattctgacttccacattccaaaagccacactcaaagatagcggctcctacttctgcagggggcttgttgggagtaaaaatgtgtcttcagagactgtgaacatcaccatcactcaaggtttggcagtgtcaaccatctcatcattctctccacctggcgcggatccaccaagggcctctgccctccctgccccaccgacaggctccgccctccctgacccgcagacagcctctgccctccctgacccgccagcagcctctgccctccctgcggccctggcggtgatctccttcctcctcgggctgggcctgggggtggcgtgtgtgctggcgaggacgcgtgttattctccgctggcgctaccacgccttgcgtggagagctgtaccggccggcctgggagccccaggactacgagatggtggagttgttcctgcgcaggctgcgcctctggatgggcctcagcaaggtcaaggagttccgccacaaagtccgctttgaagggatggagccgctgccctctcgctcctccaggggctccaaggtatccccggatgtgcccccacccagcgctggctccgatgcctcgcacccctccacctcctccagccagctggatgggctgagcgtgagcctgggccggtag

SEQ ID NO: 40 - protein, 367 aa, synthetic construct
MWQLLLPTALLLLVSAGMRTEDLPKAVVFLEPQWYSVLEKDSVTLKCQGAYSPEDNSTQWFHNESLISSQASSYFIDAATVNDSGEYRCQTNLSTLSDPVQLEVHIGWLLLQAPRWVFKEEDPIHLRCHSWKNTALHKVTYLQNGKDRKYFHHNSDFHIPKATLKDSGSYFCRGLVGSKNVSSETVNITITQGLAVSTISSFSPPGADPPRASALPAPPTGSALPDPQTASALPDPPAASALPAALAVISFLLGLGLGVACVLARTRRFEGMEPLPSRSSRGSKVSPDVPPPSAGSDASHPSTSSSQLDGLSVSLGRLGTRCEPEPSRLQAVFEALLTQFDRLNQATEDVYQLEQQLHSLQGRRSSR

SEQ ID NO: 41 - DNA, 1104 bp, synthetic construct
  source 1..1104: mol_type = other DNA
atgtggcagctgctcctcccaactgctctgctacttctagtttcagctggcatgcggactgaagatctcccaaaggctgtggtgttcctggagcctcaatggtacagcgtgcttgagaaggacagtgtgactctgaagtgccagggagcctactcccctgaggacaattccacacagtggtttcacaatgagagcctcatctcaagccaggcctcgagctacttcattgacgctgccacagtcaacgacagtggagagtacaggtgccagacaaacctctccaccctcagtgacccggtgcagctagaagtccatatcggctggctgttgctccaggcccctcggtgggtgttcaaggaggaagaccctattcacctgaggtgtcacagctggaagaacactgctctgcataaggtcacatatttacagaatggcaaagacaggaagtattttcatcataattctgacttccacattccaaaagccacactcaaagatagcggctcctacttctgcagggggcttgttgggagtaaaaatgtgtcttcagagactgtgaacatcaccatcactcaaggtttggcagtgtcaaccatctcatcattctctccacctggcgcggatccaccaagggcctctgccctccctgccccaccgacaggctccgccctccctgacccgcagacagcctctgccctccctgacccgccagcagcctctgccctccctgcggccctggcggtgatctccttcctcctcgggctgggcctgggggtggcgtgtgtgctggcgaggacgcgtcgctttgaagggatggagccgctgccctctcgctcctccaggggctccaaggtatccccggatgtgcccccacccagcgctggctccgatgcctcgcacccctccacctcctccagccagctggatgggctgagcgtgagcctgggccggctggggacaaggtgtgagcctgagccctcccgcctccaagccgtgttcgaggccctgctcacccagtttgaccgactcaaccaggccacagaggacgtctaccagctggagcagcagctgcacagcctgcaaggccgcaggagcagccggtag

SEQ ID NO: 42 - protein, 357 aa, synthetic construct
MWQLLLPTALLLLVSAGMRTEDLPKAVVFLEPQWYSVLEKDSVTLKCQGAYSPEDNSTQWFHNESLISSQASSYFIDAATVNDSGEYRCQTNLSTLSDPVQLEVHIGWLLLQAPRWVFKEEDPIHLRCHSWKNTALHKVTYLQNGKDRKYFHHNSDFHIPKATLKDSGSYFCRGLVGSKNVSSETVNITITQGLAVSTISSFSPPGADPPRASALPAPPTGSALPDPQTASALPDPPAASALPAALAVISFLLGLGLGVACVLARTRRFEGMEPLPSRSSRGSKVSPDVPPPSAGSDASHPSTSSSQLDGLSVSLGRLGTRCEPEPSRLQAVFEALLTQFDRLNQATEDVYQLEQQL

SEQ ID NO: 43 - DNA, 1074 bp, synthetic construct
  source 1..1074: mol_type = other DNA
atgtggcagctgctcctcccaactgctctgctacttctagtttcagctggcatgcggactgaagatctcccaaaggctgtggtgttcctggagcctcaatggtacagcgtgcttgagaaggacagtgtgactctgaagtgccagggagcctactcccctgaggacaattccacacagtggtttcacaatgagagcctcatctcaagccaggcctcgagctacttcattgacgctgccacagtcaacgacagtggagagtacaggtgccagacaaacctctccaccctcagtgacccggtgcagctagaagtccatatcggctggctgttgctccaggcccctcggtgggtgttcaaggaggaagaccctattcacctgaggtgtcacagctggaagaacactgctctgcataaggtcacatatttacagaatggcaaagacaggaagtattttcatcataattctgacttccacattccaaaagccacactcaaagatagcggctcctacttctgcagggggcttgttgggagtaaaaatgtgtcttcagagactgtgaacatcaccatcactcaaggtttggcagtgtcaaccatctcatcattctctccacctggcgcggatccaccaagggcctctgccctccctgccccaccgacaggctccgccctccctgacccgcagacagcctctgccctccctgacccgccagcagcctctgccctccctgcggccctggcggtgatctccttcctcctcgggctgggcctgggggtggcgtgtgtgctggcgaggacgcgtcgctttgaagggatggagccgctgccctctcgctcctccaggggctccaaggtatccccggatgtgcccccacccagcgctggctccgatgcctcgcacccctccacctcctccagccagctggatgggctgagcgtgagcctgggccggctggggacaaggtgtgagcctgagccctcccgcctccaagccgtgttcgaggccctgctcacccagtttgaccgactcaaccaggccacagaggacgtctaccagctggagcagcagctgtag

SEQ ID NO: 44 - protein, 378 aa, synthetic construct
MWQLLLPTALLLLVSAGMRTEDLPKAVVFLEPQWYSVLEKDSVTLKCQGAYSPEDNSTQWFHNESLISSQASSYFIDAATVNDSGEYRCQTNLSTLSDPVQLEVHIGWLLLQAPRWVFKEEDPIHLRCHSWKNTALHKVTYLQNGKDRKYFHHNSDFHIPKATLKDSGSYFCRGLVGSKNVSSETVNITITQGLAVSTISSFSPPGADPPRASALPAPPTGSALPDPQTASALPDPPAASALPAALAVISFLLGLGLGVACVLARTRQLDGLSVSLGRLGTRCEPEPSRLQAVFEALLTQFDRLNQATEDVYQLEQQLHSLQGRRSSRAPAGSSRGPSPGLRPALPSRLARASRGVDLATGPSRTPLRAKNKVHPSST

SEQ ID NO: 45 - DNA, 1137 bp, synthetic construct
  source 1..1137: mol_type = other DNA
atgtggcagctgctcctcccaactgctctgctacttctagtttcagctggcatgcggactgaagatctcccaaaggctgtggtgttcctggagcctcaatggtacagcgtgcttgagaaggacagtgtgactctgaagtgccagggagcctactcccctgaggacaattccacacagtggtttcacaatgagagcctcatctcaagccaggcctcgagctacttcattgacgctgccacagtcaacgacagtggagagtacaggtgccagacaaacctctccaccctcagtgacccggtgcagctagaagtccatatcggctggctgttgctccaggcccctcggtgggtgttcaaggaggaagaccctattcacctgaggtgtcacagctggaagaacactgctctgcataaggtcacatatttacagaatggcaaagacaggaagtattttcatcataattctgacttccacattccaaaagccacactcaaagatagcggctcctacttctgcagggggcttgttgggagtaaaaatgtgtcttcagagactgtgaacatcaccatcactcaaggtttggcagtgtcaaccatctcatcattctctccacctggcgcggatccaccaagggcctctgccctccctgccccaccgacaggctccgccctccctgacccgcagacagcctctgccctccctgacccgccagcagcctctgccctccctgcggccctggcggtgatctccttcctcctcgggctgggcctgggggtggcgtgtgtgctggcgaggacgcgtcagctggatgggctgagcgtgagcctgggccggctggggacaaggtgtgagcctgagccctcccgcctccaagccgtgttcgaggccctgctcacccagtttgaccgactcaaccaggccacagaggacgtctaccagctggagcagcagctgcacagcctgcaaggccgcaggagcagccgggcgcccgccggatcttcccgtggcccatccccgggcctgcggccagcactgcccagccgccttgcccgggccagtcggggtgtggacctggccactggccccagcaggacaccccttcgggccaagaacaaggtccaccccagcagcacttag

SEQ ID NO: 46 - protein, 367 aa, synthetic construct
MWQLLLPTALLLLVSAGMRTEDLPKAVVFLEPQWYSVLEKDSVTLKCQGAYSPEDNSTQWFHNESLISSQASSYFIDAATVNDSGEYRCQTNLSTLSDPVQLEVHIGWLLLQAPRWVFKEEDPIHLRCHSWKNTALHKVTYLQNGKDRKYFHHNSDFHIPKATLKDSGSYFCRGLVGSKNVSSETVNITITQGLAVSTISSFSPPGADPPRASALPAPPTGSALPDPQTASALPDPPAASALPAALAVISFLLGLGLGVACVLARTRLGTRCEPEPSRLQAVFEALLTQFDRLNQATEDVYQLEQQLHSLQGRRSSRAPAGSSRGPSPGLRPALPSRLARASRGVDLATGPSRTPLRAKNKVHPSST

SEQ ID NO: 47 - DNA, 1104 bp, synthetic construct
  source 1..1104: mol_type = other DNA
atgtggcagctgctcctcccaactgctctgctacttctagtttcagctggcatgcggactgaagatctcccaaaggctgtggtgttcctggagcctcaatggtacagcgtgcttgagaaggacagtgtgactctgaagtgccagggagcctactcccctgaggacaattccacacagtggtttcacaatgagagcctcatctcaagccaggcctcgagctacttcattgacgctgccacagtcaacgacagtggagagtacaggtgccagacaaacctctccaccctcagtgacccggtgcagctagaagtccatatcggctggctgttgctccaggcccctcggtgggtgttcaaggaggaagaccctattcacctgaggtgtcacagctggaagaacactgctctgcataaggtcacatatttacagaatggcaaagacaggaagtattttcatcataattctgacttccacattccaaaagccacactcaaagatagcggctcctacttctgcagggggcttgttgggagtaaaaatgtgtcttcagagactgtgaacatcaccatcactcaaggtttggcagtgtcaaccatctcatcattctctccacctggcgcggatccaccaagggcctctgccctccctgccccaccgacaggctccgccctccctgacccgcagacagcctctgccctccctgacccgccagcagcctctgccctccctgcggccctggcggtgatctccttcctcctcgggctgggcctgggggtggcgtgtgtgctggcgaggacgcgtctggggacaaggtgtgagcctgagccctcccgcctccaagccgtgttcgaggccctgctcacccagtttgaccgactcaaccaggccacagaggacgtctaccagctggagcagcagctgcacagcctgcaaggccgcaggagcagccgggcgcccgccggatcttcccgtggcccatccccgggcctgcggccagcactgcccagccgccttgcccgggccagtcggggtgtggacctggccactggccccagcaggacaccccttcgggccaagaacaaggtccaccccagcagcacttag

SEQ ID NO: 48 - protein, 317 aa, synthetic construct
MWQLLLPTALLLLVSAGMRTEDLPKAVVFLEPQWYSVLEKDSVTLKCQGAYSPEDNSTQWFHNESLISSQASSYFIDAATVNDSGEYRCQTNLSTLSDPVQLEVHIGWLLLQAPRWVFKEEDPIHLRCHSWKNTALHKVTYLQNGKDRKYFHHNSDFHIPKATLKDSGSYFCRGLVGSKNVSSETVNITITQGLAVSTISSFSPPGADPPRASALPAPPTGSALPDPQTASALPDPPAASALPAALAVISFLLGLGLGVACVLARTRLGTRCEPEPSRLQAVFEALLTQFDRLNQATEDVYQLEQQLHSLQGRRSSR

SEQ ID NO: 49 - DNA, 954 bp, synthetic construct
  source 1..954: mol_type = other DNA
atgtggcagctgctcctcccaactgctctgctacttctagtttcagctggcatgcggactgaagatctcccaaaggctgtggtgttcctggagcctcaatggtacagcgtgcttgagaaggacagtgtgactctgaagtgccagggagcctactcccctgaggacaattccacacagtggtttcacaatgagagcctcatctcaagccaggcctcgagctacttcattgacgctgccacagtcaacgacagtggagagtacaggtgccagacaaacctctccaccctcagtgacccggtgcagctagaagtccatatcggctggctgttgctccaggcccctcggtgggtgttcaaggaggaagaccctattcacctgaggtgtcacagctggaagaacactgctctgcataaggtcacatatttacagaatggcaaagacaggaagtattttcatcataattctgacttccacattccaaaagccacactcaaagatagcggctcctacttctgcagggggcttgttgggagtaaaaatgtgtcttcagagactgtgaacatcaccatcactcaaggtttggcagtgtcaaccatctcatcattctctccacctggcgcggatccaccaagggcctctgccctccctgccccaccgacaggctccgccctccctgacccgcagacagcctctgccctccctgacccgccagcagcctctgccctccctgcggccctggcggtgatctccttcctcctcgggctgggcctgggggtggcgtgtgtgctggcgaggacgcgtctggggacaaggtgtgagcctgagccctcccgcctccaagccgtgttcgaggccctgctcacccagtttgaccgactcaaccaggccacagaggacgtctaccagctggagcagcagctgcacagcctgcaaggccgcaggagcagccggtag

SEQ ID NO: 50 - protein, 317 aa, synthetic construct
MWQLLLPTALLLLVSAGMRTEDLPKAVVFLEPQWYSVLEKDSVTLKCQGAYSPEDNSTQWFHNESLISSQASSYFIDAATVNDSGEYRCQTNLSTLSDPVQLEVHIGWLLLQAPRWVFKEEDPIHLRCHSWKNTALHKVTYLQNGKDRKYFHHNSDFHIPKATLKDSGSYFCRGLVGSKNVSSETVNITITQGLAVSTISSFSPPGADPPRASALPAPPTGSALPDPQTASALPDPPAASALPAALAVISFLLGLGLGVACVLARTRAPAGSSRGPSPGLRPALPSRLARASRGVDLATGPSRTPLRAKNKVHPSST

SEQ ID NO: 51 - DNA, 954 bp, synthetic construct
  source 1..954: mol_type = other DNA
atgtggcagctgctcctcccaactgctctgctacttctagtttcagctggcatgcggactgaagatctcccaaaggctgtggtgttcctggagcctcaatggtacagcgtgcttgagaaggacagtgtgactctgaagtgccagggagcctactcccctgaggacaattccacacagtggtttcacaatgagagcctcatctcaagccaggcctcgagctacttcattgacgctgccacagtcaacgacagtggagagtacaggtgccagacaaacctctccaccctcagtgacccggtgcagctagaagtccatatcggctggctgttgctccaggcccctcggtgggtgttcaaggaggaagaccctattcacctgaggtgtcacagctggaagaacactgctctgcataaggtcacatatttacagaatggcaaagacaggaagtattttcatcataattctgacttccacattccaaaagccacactcaaagatagcggctcctacttctgcagggggcttgttgggagtaaaaatgtgtcttcagagactgtgaacatcaccatcactcaaggtttggcagtgtcaaccatctcatcattctctccacctggcgcggatccaccaagggcctctgccctccctgccccaccgacaggctccgccctccctgacccgcagacagcctctgccctccctgacccgccagcagcctctgccctccctgcggccctggcggtgatctccttcctcctcgggctgggcctgggggtggcgtgtgtgctggcgaggacgcgtgcgcccgccggatcttcccgtggcccatccccgggcctgcggccagcactgcccagccgccttgcccgggccagtcggggtgtggacctggccactggccccagcaggacaccccttcgggccaagaacaaggtccaccccagcagcacttag

SEQ ID NO: 52 - protein, 290 aa, synthetic construct
MLGIWTLLPLVLTSVARLSSKSVNAQVTDINSKGLELRKTVTTVETQNLEGLHHDGQFCHKPCPPGERKARDCTVNGDEPDCVPCQEGKEYTDKAHFSSKCRRCRLCDEGHGLEVEINCTRTQNTKCRCKPNFFCNSTVCEHCDPCTKCEHGIIKECTLTSNTKCKEEGSRSNLGWLCLLLLPIPLIVWVLGTRCEPEPSRLQAVFEALLTQFDRLNQATEDVYQLEQQLHSLQGRRSSRAPAGSSRGPSPGLRPALPSRLARASRGVDLATGPSRTPLRAKNKVHPSST

SEQ ID NO: 53 - DNA, 873 bp, synthetic construct
  source 1..873: mol_type = other DNA
atgctgggcatctggaccctcctacctctggttcttacgtctgttgctagattatcgtccaaaagtgttaatgcccaagtgactgacatcaactccaagggattggaattgaggaagactgttactacagttgagactcagaacttggaaggcctgcatcatgatggccaattctgccataagccctgtcctccaggtgaaaggaaagctagggactgcacagtcaatggggatgaaccagactgcgtgccctgccaagaagggaaggagtacacagacaaagcccatttttcttccaaatgcagaagatgtagattgtgtgatgaaggacatggcttagaagtggaaataaactgcacccggacccagaataccaagtgcagatgtaaaccaaactttttttgtaactctactgtatgtgaacactgtgacccttgcaccaaatgtgaacatggaatcatcaaggaatgcacactcaccagcaacaccaagtgcaaagaggaaggatccagatctaacttggggtggctttgtcttcttcttttgccaattccactaattgtttgggtgctggggacaaggtgtgagcctgagccctcccgcctccaagccgtgttcgaggccctgctcacccagtttgaccgactcaaccaggccacagaggacgtctaccagctggagcagcagctgcacagcctgcaaggccgcaggagcagccgggcgcccgccggatcttcccgtggcccatccccgggcctgcggccagcactgcccagccgccttgcccgggccagtcggggtgtggacctggccactggccccagcaggacaccccttcgggccaagaacaaggtccaccccagcagcacttaa

SEQ ID NO: 54 - protein, 240 aa, synthetic construct
MLGIWTLLPLVLTSVARLSSKSVNAQVTDINSKGLELRKTVTTVETQNLEGLHHDGQFCHKPCPPGERKARDCTVNGDEPDCVPCQEGKEYTDKAHFSSKCRRCRLCDEGHGLEVEINCTRTQNTKCRCKPNFFCNSTVCEHCDPCTKCEHGIIKECTLTSNTKCKEEGSRSNLGWLCLLLLPIPLIVWVLGTRCEPEPSRLQAVFEALLTQFDRLNQATEDVYQLEQQLHSLQGRRSSR

SEQ ID NO: 55 - DNA, 723 bp, synthetic construct
  source 1..723: mol_type = other DNA
atgctgggcatctggaccctcctacctctggttcttacgtctgttgctagattatcgtccaaaagtgttaatgcccaagtgactgacatcaactccaagggattggaattgaggaagactgttactacagttgagactcagaacttggaaggcctgcatcatgatggccaattctgccataagccctgtcctccaggtgaaaggaaagctagggactgcacagtcaatggggatgaaccagactgcgtgccctgccaagaagggaaggagtacacagacaaagcccatttttcttccaaatgcagaagatgtagattgtgtgatgaaggacatggcttagaagtggaaataaactgcacccggacccagaataccaagtgcagatgtaaaccaaactttttttgtaactctactgtatgtgaacactgtgacccttgcaccaaatgtgaacatggaatcatcaaggaatgcacactcaccagcaacaccaagtgcaaagaggaaggatccagatctaacttggggtggctttgtcttcttcttttgccaattccactaattgtttgggtgctggggacaaggtgtgagcctgagccctcccgcctccaagccgtgttcgaggccctgctcacccagtttgaccgactcaaccaggccacagaggacgtctaccagctggagcagcagctgcacagcctgcaaggccgcaggagcagccggtag

SEQ ID NO: 56 - protein, 10 aa, synthetic construct
FEGMEPLPSR

SEQ ID NO: 57 - protein, 14 aa, synthetic construct
LQAVFEALLTQFDR

SEQ ID NO: 58 - protein, 12 aa, synthetic construct
EVLAASDAALLR

SEQ ID NO: 59 - protein, 9 aa, synthetic construct
SDLFLDDSK

SEQ ID NO: 60 - protein, 7 aa, synthetic construct
NSLDIFR